European Patent Application EP 4 755 389 A1, published June 10, 2026. Title: 融合多肽、包含其编码基因的表达盒、基因递送载体、药物组合物及用途. Applicant: 北京因诺惟康医药科技有限公司. The sequence listing filed with the application follows.

SEQUENCE LISTING (111 sequences)

SEQ ID NO: 1 - protein, 452 aa, synthetic construct
MYRMQLLSCIALSLALVTNSSDTGRPFVEMYSEIPEIIHMTEGRELVIPCRVTSPNITVTLKKFPLDTLIPDGKRIIWDSRKGFIISNATYKEIGLLTCEATVNGHLYKTNYLTHRQTNTIIDVVLSPSHGIELSVGEKLVLNCTARTELNVGIDFNWEYPSSKHQHKKLVNRDLKTQSGSEMKKFLSTLTIDGVTRSDQGLYTCAASSGLMTKKNSTFVRVHEKDKTHTCPPCPAPELLGGPSVFLFPPKPKDTLMISRTPEVTCVVVDVSHEDPEVKFNWYVDGVEVHNAKTKPREEQYNSTYRVVSVLTVLHQDWLNGKEYKCKVSNKALPAPIEKTISKAKGQPREPQVYTLPPSRDELTKNQVSLTCLVKGFYPSDIAVEWESNGQPENNYKTTPPVLDSDGSFFLYSKLTVDKSRWQQGNVFSCSVMHEALHNHYTQKSLSLSPGK

SEQ ID NO: 2 - DNA, 1359 bp, synthetic construct
  source 1..1359: mol_type = other DNA
atgtacagaatgcagctgctgagctgcatagccctgtctctggccctggtgaccaacagctctgacacaggcagaccctttgtggaaatgtactctgagatccctgagatcatccacatgacagagggcagagagctggtcatcccctgcagagtgacaagccccaacatcacagtgaccctgaagaagttccctctggacacactgatccctgatggcaagagaatcatctgggacagcagaaagggcttcatcatcagcaatgccacctacaaagagattggcctgctgacctgtgaagccacagtgaatggccacctgtacaagaccaactacctgacacacagacagaccaacaccatcattgatgtggtgctgagccccagccatggcattgagctgtctgtgggagagaagctggtgctgaactgcacagccagaacagagctgaatgtgggcattgacttcaactgggagtaccccagcagcaagcaccagcacaagaaactggtcaacagggacctgaaaacccagagtggctctgagatgaagaaattcctgagcaccctgaccattgatggggtcaccagatctgaccagggcctgtacacatgtgctgccagctctggactgatgaccaagaaaaacagcacctttgtcagagtgcatgagaaggacaagacccacacctgtcctccatgtcctgcacctgagctgcttggaggcccctctgtgttcctgtttcctccaaagcctaaggacaccctgatgatcagcagaacacctgaagtgacctgtgtggtggtggatgtgtcccatgaggacccagaagtgaagttcaattggtatgtggatggggttgaagtgcacaatgccaagaccaagcctagagaggaacagtacaactccacctacagagtggtgtcagtgctgacagtgctgcaccaggactggctgaatggcaaagagtacaagtgcaaggtgtccaacaaggccctgcctgctcctattgagaaaaccatctccaaggccaagggccagcctagggaaccccaggtttacacactgccacctagcagggatgagctgacaaagaaccaggtgtccctgacctgcctggtcaagggcttctacccctctgacattgctgtggaatgggagagcaatggccagcctgagaacaactacaagacaacccctcctgtgctggactctgatggctcattcttcctgtacagcaagctgactgtggacaagagcagatggcagcagggaaatgtgttcagctgctctgtgatgcatgaggccctgcacaaccactacacccagaaaagcctgagcctgtctcctggcaagtga

SEQ ID NO: 3 - DNA, 874 bp, synthetic construct
  source 1..874: mol_type = other DNA
acgcgtctagttattaatagtaatcaattacggggtcattagttcatagcccatatatggagttccgcgttacataacttacggtaaatggcccgcctggctgaccgcccaacgacccccgcccattgacgtcaataatgacgtatgttcccatagtaacgccaatagggactttccattgacgtcaatgggtggagtatttacggtaaactgcccacttggcagtacatcaagtgtatcatatgccaagtacgccccctattgacgtcaatgacggtaaatggcccgcctggcattatgcccagtacatgaccttacgggactttcctacttggcagtacatctacgtattagtcatcgctattaccatggtcgaggtgagccccacgttctgcttcactctccccatctcccccccctccccacccccaattttgtatttatttattttttaattattttgtgcagcgatgggggcggggggggggggggcgcgcgccaggcggggcggggcggggcgaggggcggggcggggcgaggcggagaggtgcggcggcagccaatcagagcggcgcgctccgaaagtttccttttatggcgaggcggcggcggcggcggccctataaaaagcgaagcgcgcggcgggcggggagtcgctgcgttgccttcgccccgtgccccgctccgcgccgcctcgcgccgcccgccccggctctgactgaccgcgttactcccacaggtgagcgggcgggacggcccttctcctccgggctgtaattagcaagaggtaagggtttaagggatggttggttggtggggtattaatgtttaattacctgttttacaggcctgaaatcacttggttttaggttgg

SEQ ID NO: 4 - DNA, 1714 bp, synthetic construct
  source 1..1714: mol_type = other DNA
acgcgtctagttattaatagtaatcaattacggggtcattagttcatagcccatatatggagttccgcgttacataacttacggtaaatggcccgcctggctgaccgcccaacgacccccgcccattgacgtcaataatgacgtatgttcccatagtaacgccaatagggactttccattgacgtcaatgggtggagtatttacggtaaactgcccacttggcagtacatcaagtgtatcatatgccaagtacgccccctattgacgtcaatgacggtaaatggcccgcctggcattatgcccagtacatgaccttacgggactttcctacttggcagtacatctacgtattagtcatcgctattaccatggtcgaggtgagccccacgttctgcttcactctccccatctcccccccctccccacccccaattttgtatttatttattttttaattattttgtgcagcgatgggggcggggggggggggggcgcgcgccaggcggggcggggcggggcgaggggcggggcggggcgaggcggagaggtgcggcggcagccaatcagagcggcgcgctccgaaagtttccttttatggcgaggcggcggcggcggcggccctataaaaagcgaagcgcgcggcgggcgggagtcgctgcgcgctgccttcgccccgtgccccgctccgccgccgcctcgcgccgcccgccccggctctgactgaccgcgttactcccacaggtgagcgggcgggacggcccttctcctccgggctgtaattagcgcttggtttaatgacggcttgtttcttttctgtggctgcgtgaaagccttgaggggctccgggagggccctttgtgcggggggagcggctcggggggtgcgtgcgtgtgtgtgtgcgtggggagcgccgcgtgcggctccgcgctgcccggcggctgtgagcgctgcgggcgcggcgcggggctttgtgcgctccgcagtgtgcgcgaggggagcgcggccgggggcggtgccccgcggtgcggggggggctgcgaggggaacaaaggctgcgtgcggggtgtgtgcgtgggggggtgagcagggggtgtgggcgcgtcggtcgggctgcaaccccccctgcacccccctccccgagttgctgagcacggcccggcttcgggtgcggggctccgtacggggcgtggcgcggggctcgccgtgccgggcggggggtggcggcaggtgggggtgccgggcggggcggggccgcctcgggccggggagggctcgggggaggggcgcggcggcccccggagcgccggcggctgtcgaggcgcggcgagccgcagccattgccttttatggtaatcgtgcgagagggcgcagggacttcctttgtcccaaatctgtgcggagccgaaatctgggaggcgccgccgcaccccctctagcgggcgcggggcgaagcggtgcggcgccggcaggaaggaaatgggcggggagggccttcgtgcgtcgccgcgccgccgtccccttctccctctccagcctcggggctgtccgcggggggacggctgccttcgggggggacggggcagggcggggttcggcttctggcgtgtgaccggcggctctagagcctctgctaaccatgttcatgccttcttctttttcctacagctcctgggcaacgtgctggttattgtgctgtctcatcattttggcaaag

SEQ ID NO: 5 - DNA, 660 bp, synthetic construct
  source 1..660: mol_type = other DNA
acgcgtctagttattaatagtaatcaattacggggtcattagttcatagcccatatatggagttccgcgttacataacttacggtaaatggcccgcctggctgaccgcccaacgacccccgcccattgacgtcaataatgacgtatgttcccatagtaacgccaatagggactttccattgacgtcaatgggtggagtatttacggtaaactgcccacttggcagtacatcaagtgtatcatatgccaagtacgccccctattgacgtcaatgacggtaaatggcccgcctggcattatgcccagtacatgaccttatgggactttcctacttggcagtacatctacgtattagtcatcgctattaccatggtgatgcggttttggcagtacatcaatgggcgtggatagcggtttgactcacggggatttccaagtctccaccccattgacgtcaatgggagtttgttttggcaccaaaatcaacgggactttccaaaatgtcgtaacaactccgccccattgacgcaaatgggcggtaggcgtgtacggtgggaggtctatataagcagagctcgtttagtgaaccgtcagatcgcctggagacgccatccacgctgttttgacctccatagaagacaccgggaccgatccagcctcc

SEQ ID NO: 6 - DNA, 493 bp, synthetic construct
  source 1..493: mol_type = other DNA
cgaatcccggccgggaacggtgcattggaacgcggattccccgtgccaagagtgacgtaagtaccgcctatagagtctataggcccacaaaaaatgctttcttcttttaatatacttttttgtttatcttatttctaatactttccctaatctctttctttcagggcaataatgatacaatgtatcatgcctctttgcaccattctaaagaataacagtgataatttctgggttaaggcaatagcaatatttctgcatataaatatttctgcatataaattgtaactgatgtaagaggtttcatattgctaatagcagctacaatccagctaccattctgcttttattttatggttgggataaggctggattattctgagtccaagctaggcccttttgctaatcatgttcatacctcttatcttcctcccacagctcctgggcaacgtgctggtctgtgtgctggcccatcactttggcaaagaattgggat

SEQ ID NO: 7 - DNA, 481 bp, synthetic construct
  source 1..481: mol_type = other DNA
cgggtggcatccctgtgacccctccccagtgcctctcctggccctggaagttgccactccagtgcccaccagccttgtcctaataaaattaagttgcatcattttgtctgactaggtgtccttctataatattatggggtggaggggggtggtatggagcaaggggcaagttgggaagacaacctgtagggcctgcggggtctattgggaaccaagctggagtgcagtggcacaatcttggctcactgcaatctccgcctcctgggttcaagcgattctcctgcctcagcctcccgagttgttgggattccaggcatgcatgaccaggctcagctaatttttgtttttttggtagagacggggtttcaccatattggccaggctggtctccaactcctaatctcaggtgatctacccaccttggcctcccaaattgctgggattacaggcgtgaaccactgctcccttccctgtccttcgg

SEQ ID NO: 8 - DNA, 3032 bp, synthetic construct
  source 1..3032: mol_type = other DNA
acgcgtctagttattaatagtaatcaattacggggtcattagttcatagcccatatatggagttccgcgttacataacttacggtaaatggcccgcctggctgaccgcccaacgacccccgcccattgacgtcaataatgacgtatgttcccatagtaacgccaatagggactttccattgacgtcaatgggtggagtatttacggtaaactgcccacttggcagtacatcaagtgtatcatatgccaagtacgccccctattgacgtcaatgacggtaaatggcccgcctggcattatgcccagtacatgaccttatgggactttcctacttggcagtacatctacgtattagtcatcgctattaccatggtgatgcggttttggcagtacatcaatgggcgtggatagcggtttgactcacggggatttccaagtctccaccccattgacgtcaatgggagtttgttttggcaccaaaatcaacgggactttccaaaatgtcgtaacaactccgccccattgacgcaaatgggcggtaggcgtgtacggtgggaggtctatataagcagagctcgtttagtgaaccgtcagatcgcctggagacgccatccacgctgttttgacctccatagaagacaccgggaccgatccagcctccgcggattcgaatcccggccgggaacggtgcattggaacgcggattccccgtgccaagagtgacgtaagtaccgcctatagagtctataggcccacaaaaaatgctttcttcttttaatatacttttttgtttatcttatttctaatactttccctaatctctttctttcagggcaataatgatacaatgtatcatgcctctttgcaccattctaaagaataacagtgataatttctgggttaaggcaatagcaatatttctgcatataaatatttctgcatataaattgtaactgatgtaagaggtttcatattgctaatagcagctacaatccagctaccattctgcttttattttatggttgggataaggctggattattctgagtccaagctaggcccttttgctaatcatgttcatacctcttatcttcctcccacagctcctgggcaacgtgctggtctgtgtgctggcccatcactttggcaaagaattgggataattactagatcgccaccatgtacagaatgcagctgctgagctgcatagccctgtctctggccctggtgaccaacagctctgacacaggcagaccctttgtggaaatgtactctgagatccctgagatcatccacatgacagagggcagagagctggtcatcccctgcagagtgacaagccccaacatcacagtgaccctgaagaagttccctctggacacactgatccctgatggcaagagaatcatctgggacagcagaaagggcttcatcatcagcaatgccacctacaaagagattggcctgctgacctgtgaagccacagtgaatggccacctgtacaagaccaactacctgacacacagacagaccaacaccatcattgatgtggtgctgagccccagccatggcattgagctgtctgtgggagagaagctggtgctgaactgcacagccagaacagagctgaatgtgggcattgacttcaactgggagtaccccagcagcaagcaccagcacaagaaactggtcaacagggacctgaaaacccagagtggctctgagatgaagaaattcctgagcaccctgaccattgatggggtcaccagatctgaccagggcctgtacacatgtgctgccagctctggactgatgaccaagaaaaacagcacctttgtcagagtgcatgagaaggacaagacccacacctgtcctccatgtcctgcacctgagctgcttggaggcccctctgtgttcctgtttcctccaaagcctaaggacaccctgatgatcagcagaacacctgaagtgacctgtgtggtggtggatgtgtcccatgaggacccagaagtgaagttcaattggtatgtggatggggttgaagtgcacaatgccaagaccaagcctagagaggaacagtacaactccacctacagagtggtgtcagtgctgacagtgctgcaccaggactggctgaatggcaaagagtacaagtgcaaggtgtccaacaaggccctgcctgctcctattgagaaaaccatctccaaggccaagggccagcctagggaaccccaggtttacacactgccacctagcagggatgagctgacaaagaaccaggtgtccctgacctgcctggtcaagggcttctacccctctgacattgctgtggaatgggagagcaatggccagcctgagaacaactacaagacaacccctcctgtgctggactctgatggctcattcttcctgtacagcaagctgactgtggacaagagcagatggcagcagggaaatgtgttcagctgctctgtgatgcatgaggccctgcacaaccactacacccagaaaagcctgagcctgtctcctggcaagtgagcggccgcaagcttcgggtggcatccctgtgacccctccccagtgcctctcctggccctggaagttgccactccagtgcccaccagccttgtcctaataaaattaagttgcatcattttgtctgactaggtgtccttctataatattatggggtggaggggggtggtatggagcaaggggcaagttgggaagacaacctgtagggcctgcggggtctattgggaaccaagctggagtgcagtggcacaatcttggctcactgcaatctccgcctcctgggttcaagcgattctcctgcctcagcctcccgagttgttgggattccaggcatgcatgaccaggctcagctaatttttgtttttttggtagagacggggtttcaccatattggccaggctggtctccaactcctaatctcaggtgatctacccaccttggcctcccaaattgctgggattacaggcgtgaaccactgctcccttccctgtccttcgg

SEQ ID NO: 9 - DNA, 2746 bp, synthetic construct
  source 1..2746: mol_type = other DNA
acgcgtctagttattaatagtaatcaattacggggtcattagttcatagcccatatatggagttccgcgttacataacttacggtaaatggcccgcctggctgaccgcccaacgacccccgcccattgacgtcaataatgacgtatgttcccatagtaacgccaatagggactttccattgacgtcaatgggtggagtatttacggtaaactgcccacttggcagtacatcaagtgtatcatatgccaagtacgccccctattgacgtcaatgacggtaaatggcccgcctggcattatgcccagtacatgaccttacgggactttcctacttggcagtacatctacgtattagtcatcgctattaccatggtcgaggtgagccccacgttctgcttcactctccccatctcccccccctccccacccccaattttgtatttatttattttttaattattttgtgcagcgatgggggcggggggggggggggcgcgcgccaggcggggcggggcggggcgaggggcggggcggggcgaggcggagaggtgcggcggcagccaatcagagcggcgcgctccgaaagtttccttttatggcgaggcggcggcggcggcggccctataaaaagcgaagcgcgcggcgggcggggagtcgctgcgttgccttcgccccgtgccccgctccgcgccgcctcgcgccgcccgccccggctctgactgaccgcgttactcccacaggtgagcgggcgggacggcccttctcctccgggctgtaattagcaagaggtaagggtttaagggatggttggttggtggggtattaatgtttaattacctgttttacaggcctgaaatcacttggttttaggttggaattactagatcgccaccatgtacagaatgcagctgctgagctgcatagccctgtctctggccctggtgaccaacagctctgacacaggcagaccctttgtggaaatgtactctgagatccctgagatcatccacatgacagagggcagagagctggtcatcccctgcagagtgacaagccccaacatcacagtgaccctgaagaagttccctctggacacactgatccctgatggcaagagaatcatctgggacagcagaaagggcttcatcatcagcaatgccacctacaaagagattggcctgctgacctgtgaagccacagtgaatggccacctgtacaagaccaactacctgacacacagacagaccaacaccatcattgatgtggtgctgagccccagccatggcattgagctgtctgtgggagagaagctggtgctgaactgcacagccagaacagagctgaatgtgggcattgacttcaactgggagtaccccagcagcaagcaccagcacaagaaactggtcaacagggacctgaaaacccagagtggctctgagatgaagaaattcctgagcaccctgaccattgatggggtcaccagatctgaccagggcctgtacacatgtgctgccagctctggactgatgaccaagaaaaacagcacctttgtcagagtgcatgagaaggacaagacccacacctgtcctccatgtcctgcacctgagctgcttggaggcccctctgtgttcctgtttcctccaaagcctaaggacaccctgatgatcagcagaacacctgaagtgacctgtgtggtggtggatgtgtcccatgaggacccagaagtgaagttcaattggtatgtggatggggttgaagtgcacaatgccaagaccaagcctagagaggaacagtacaactccacctacagagtggtgtcagtgctgacagtgctgcaccaggactggctgaatggcaaagagtacaagtgcaaggtgtccaacaaggccctgcctgctcctattgagaaaaccatctccaaggccaagggccagcctagggaaccccaggtttacacactgccacctagcagggatgagctgacaaagaaccaggtgtccctgacctgcctggtcaagggcttctacccctctgacattgctgtggaatgggagagcaatggccagcctgagaacaactacaagacaacccctcctgtgctggactctgatggctcattcttcctgtacagcaagctgactgtggacaagagcagatggcagcagggaaatgtgttcagctgctctgtgatgcatgaggccctgcacaaccactacacccagaaaagcctgagcctgtctcctggcaagtgagcggccgcaagcttcgggtggcatccctgtgacccctccccagtgcctctcctggccctggaagttgccactccagtgcccaccagccttgtcctaataaaattaagttgcatcattttgtctgactaggtgtccttctataatattatggggtggaggggggtggtatggagcaaggggcaagttgggaagacaacctgtagggcctgcggggtctattgggaaccaagctggagtgcagtggcacaatcttggctcactgcaatctccgcctcctgggttcaagcgattctcctgcctcagcctcccgagttgttgggattccaggcatgcatgaccaggctcagctaatttttgtttttttggtagagacggggtttcaccatattggccaggctggtctccaactcctaatctcaggtgatctacccaccttggcctcccaaattgctgggattacaggcgtgaaccactgctcccttccctgtccttcgg

SEQ ID NO: 10 - DNA, 3586 bp, synthetic construct
  source 1..3586: mol_type = other DNA
acgcgtctagttattaatagtaatcaattacggggtcattagttcatagcccatatatggagttccgcgttacataacttacggtaaatggcccgcctggctgaccgcccaacgacccccgcccattgacgtcaataatgacgtatgttcccatagtaacgccaatagggactttccattgacgtcaatgggtggagtatttacggtaaactgcccacttggcagtacatcaagtgtatcatatgccaagtacgccccctattgacgtcaatgacggtaaatggcccgcctggcattatgcccagtacatgaccttacgggactttcctacttggcagtacatctacgtattagtcatcgctattaccatggtcgaggtgagccccacgttctgcttcactctccccatctcccccccctccccacccccaattttgtatttatttattttttaattattttgtgcagcgatgggggcggggggggggggggcgcgcgccaggcggggcggggcggggcgaggggcggggcggggcgaggcggagaggtgcggcggcagccaatcagagcggcgcgctccgaaagtttccttttatggcgaggcggcggcggcggcggccctataaaaagcgaagcgcgcggcgggcgggagtcgctgcgcgctgccttcgccccgtgccccgctccgccgccgcctcgcgccgcccgccccggctctgactgaccgcgttactcccacaggtgagcgggcgggacggcccttctcctccgggctgtaattagcgcttggtttaatgacggcttgtttcttttctgtggctgcgtgaaagccttgaggggctccgggagggccctttgtgcggggggagcggctcggggggtgcgtgcgtgtgtgtgtgcgtggggagcgccgcgtgcggctccgcgctgcccggcggctgtgagcgctgcgggcgcggcgcggggctttgtgcgctccgcagtgtgcgcgaggggagcgcggccgggggcggtgccccgcggtgcggggggggctgcgaggggaacaaaggctgcgtgcggggtgtgtgcgtgggggggtgagcagggggtgtgggcgcgtcggtcgggctgcaaccccccctgcacccccctccccgagttgctgagcacggcccggcttcgggtgcggggctccgtacggggcgtggcgcggggctcgccgtgccgggcggggggtggcggcaggtgggggtgccgggcggggcggggccgcctcgggccggggagggctcgggggaggggcgcggcggcccccggagcgccggcggctgtcgaggcgcggcgagccgcagccattgccttttatggtaatcgtgcgagagggcgcagggacttcctttgtcccaaatctgtgcggagccgaaatctgggaggcgccgccgcaccccctctagcgggcgcggggcgaagcggtgcggcgccggcaggaaggaaatgggcggggagggccttcgtgcgtcgccgcgccgccgtccccttctccctctccagcctcggggctgtccgcggggggacggctgccttcgggggggacggggcagggcggggttcggcttctggcgtgtgaccggcggctctagagcctctgctaaccatgttcatgccttcttctttttcctacagctcctgggcaacgtgctggttattgtgctgtctcatcattttggcaaagaattactagatcgccaccatgtacagaatgcagctgctgagctgcatagccctgtctctggccctggtgaccaacagctctgacacaggcagaccctttgtggaaatgtactctgagatccctgagatcatccacatgacagagggcagagagctggtcatcccctgcagagtgacaagccccaacatcacagtgaccctgaagaagttccctctggacacactgatccctgatggcaagagaatcatctgggacagcagaaagggcttcatcatcagcaatgccacctacaaagagattggcctgctgacctgtgaagccacagtgaatggccacctgtacaagaccaactacctgacacacagacagaccaacaccatcattgatgtggtgctgagccccagccatggcattgagctgtctgtgggagagaagctggtgctgaactgcacagccagaacagagctgaatgtgggcattgacttcaactgggagtaccccagcagcaagcaccagcacaagaaactggtcaacagggacctgaaaacccagagtggctctgagatgaagaaattcctgagcaccctgaccattgatggggtcaccagatctgaccagggcctgtacacatgtgctgccagctctggactgatgaccaagaaaaacagcacctttgtcagagtgcatgagaaggacaagacccacacctgtcctccatgtcctgcacctgagctgcttggaggcccctctgtgttcctgtttcctccaaagcctaaggacaccctgatgatcagcagaacacctgaagtgacctgtgtggtggtggatgtgtcccatgaggacccagaagtgaagttcaattggtatgtggatggggttgaagtgcacaatgccaagaccaagcctagagaggaacagtacaactccacctacagagtggtgtcagtgctgacagtgctgcaccaggactggctgaatggcaaagagtacaagtgcaaggtgtccaacaaggccctgcctgctcctattgagaaaaccatctccaaggccaagggccagcctagggaaccccaggtttacacactgccacctagcagggatgagctgacaaagaaccaggtgtccctgacctgcctggtcaagggcttctacccctctgacattgctgtggaatgggagagcaatggccagcctgagaacaactacaagacaacccctcctgtgctggactctgatggctcattcttcctgtacagcaagctgactgtggacaagagcagatggcagcagggaaatgtgttcagctgctctgtgatgcatgaggccctgcacaaccactacacccagaaaagcctgagcctgtctcctggcaagtgagcggccgcaagcttcgggtggcatccctgtgacccctccccagtgcctctcctggccctggaagttgccactccagtgcccaccagccttgtcctaataaaattaagttgcatcattttgtctgactaggtgtccttctataatattatggggtggaggggggtggtatggagcaaggggcaagttgggaagacaacctgtagggcctgcggggtctattgggaaccaagctggagtgcagtggcacaatcttggctcactgcaatctccgcctcctgggttcaagcgattctcctgcctcagcctcccgagttgttgggattccaggcatgcatgaccaggctcagctaatttttgtttttttggtagagacggggtttcaccatattggccaggctggtctccaactcctaatctcaggtgatctacccaccttggcctcccaaattgctgggattacaggcgtgaaccactgctcccttccctgtccttcgg

SEQ ID NO: 11 - protein, 12 aa, synthetic construct
AAAGNGRAHAAA

SEQ ID NO: 12 - DNA, 3050 bp, synthetic construct
  source 1..3050: mol_type = other DNA
acgcgtctagttattaatagtaatcaattacggggtcattagttcatagcccatatatggagttccgcgttacataacttacggtaaatggcccgcctggctgaccgcccaacgacccccgcccattgacgtcaataatgacgtatgttcccatagtaacgccaatagggactttccattgacgtcaatgggtggagtatttacggtaaactgcccacttggcagtacatcaagtgtatcatatgccaagtacgccccctattgacgtcaatgacggtaaatggcccgcctggcattatgcccagtacatgaccttatgggactttcctacttggcagtacatctacgtattagtcatcgctattaccatggtgatgcggttttggcagtacatcaatgggcgtggatagcggtttgactcacggggatttccaagtctccaccccattgacgtcaatgggagtttgttttggcaccaaaatcaacgggactttccaaaatgtcgtaacaactccgccccattgacgcaaatgggcggtaggcgtgtacggtgggaggtctatataagcagagctcgtttagtgaaccgtcagatcgcctggagacgccatccacgctgttttgacctccatagaagacaccgggaccgatccagcctccgcggattcgaatcccggccgggaacggtgcattggaacgcggattccccgtgccaagagtgacgtaagtaccgcctatagagtctataggcccacaaaaaatgctttcttcttttaatatacttttttgtttatcttatttctaatactttccctaatctctttctttcagggcaataatgatacaatgtatcatgcctctttgcaccattctaaagaataacagtgataatttctgggttaaggcaatagcaatatttctgcatataaatatttctgcatataaattgtaactgatgtaagaggtttcatattgctaatagcagctacaatccagctaccattctgcttttattttatggttgggataaggctggattattctgagtccaagctaggcccttttgctaatcatgttcatacctcttatcttcctcccacagctcctgggcaacgtgctggtctgtgtgctggcccatcactttggcaaagaattgggataattactagatcgccaccatggtgtcatactgggatactggagtcttgctttgtgccctgctgtcctgcctcctcctgactggctccagctcgggctctgatacaggcagaccctttgtggaaatgtactctgagattcctgaaatcatccacatgacagagggcagagaactggtgatcccatgcagagtgaccagccctaacatcacagtgacactgaagaagttcccactggacaccctgatccctgatggaaaaagaatcatttgggacagcaggaagggctttatcatcagtaatgccacctacaaagagataggcctgctcacatgtgaagctacagtgaatggccacctgtataaaacaaactacctgacccatagacagaccaataccatcatagatgtggtgctgagccccagccatggaatagagctgtctgtgggggagaagctggtactgaactgcactgccagaactgagcttaatgtgggcatagacttcaattgggagtaccccagctccaagcaccaacacaagaagctggtcaacagggacctgaagacccagagtggctctgaaatgaaaaagtttctgagcaccctgacaatagatggtgttacaaggagtgatcagggcctgtacacctgtgcagcttctagtggcctgatgaccaaaaagaacagcacctttgtgagggtgcatgagaaggacaagacacatacctgccctccatgtcctgcccctgaactgctgggaggacctagtgtgtttctgttcccccccaagcctaaggacaccctgatgatcagcaggacccctgaggtgacatgtgtggtggtggatgtgtctcatgaggacccagaggtgaagttcaactggtatgtggatggggtggaagtgcacaatgccaaaaccaagcccagagaggaacagtacaacagcacatacagggtggtgtctgtgctgacagtcctgcaccaggattggctgaatggaaaggaatacaagtgcaaggtgtccaacaaggccctgcctgctcctatagagaagaccatcagcaaggccaagggccagcctagagagcctcaggtgtacaccctgcctccctccagagatgagctgacaaagaaccaggtgtccctgacttgcctggtcaagggcttctaccctagtgacatagcagtggaatgggaaagcaatggccaacctgagaacaactacaagacaacccccccagtgttggattcagatggcagcttcttcctgtacagcaagctgacagtggacaaaagcaggtggcagcagggcaatgtgttcagctgcagtgtgatgcatgaggccctgcacaatcactacacacagaaaagcctgagcctgtctcctggcaaatgagcggccgcaagcttcgggtggcatccctgtgacccctccccagtgcctctcctggccctggaagttgccactccagtgcccaccagccttgtcctaataaaattaagttgcatcattttgtctgactaggtgtccttctataatattatggggtggaggggggtggtatggagcaaggggcaagttgggaagacaacctgtagggcctgcggggtctattgggaaccaagctggagtgcagtggcacaatcttggctcactgcaatctccgcctcctgggttcaagcgattctcctgcctcagcctcccgagttgttgggattccaggcatgcatgaccaggctcagctaatttttgtttttttggtagagacggggtttcaccatattggccaggctggtctccaactcctaatctcaggtgatctacccaccttggcctcccaaattgctgggattacaggcgtgaaccactgctcccttccctgtccttcgg

SEQ ID NO: 13 - DNA, 7493 bp, synthetic construct
  source 1..7493: mol_type = other DNA
gcgcgccgatatcttcaaacctcccgcttcaaaatggagaccctgcgtgctcactcgggcccccccccccagcgtgaccacatggtgtcgcaaaatgtcgcaaaacactcacgtgacctctaatacaggacctccctaaccctatgacgtaattcacgtcacgactccacccctccgttaacgccccgcgccggccgctctagaactagtggatcccccggaagatcagaagttcctattccgaagttcctattctctagaaagtataggaacttctgatctgcgcagccgccatgccggggttttacgagattgtgattaaggtccccagcgaccttgacgagcatctgcccggcatttctgacagctttgtgaactgggtggccgagaaggaatgggagttgccgccagattctgacatggatctgaatctgattgagcaggcacccctgaccgtggccgagaagctgcagcgcgactttctgacggaatggcgccgtgtgagtaaggccccggaggcccttttctttgtgcaatttgagaagggagagagctacttccacatgcacgtgctcgtggaaaccaccggggtgaaatccatggttttgggacgtttcctgagtcagattcgcgaaaaactgattcagagaatttaccgcgggatcgagccgactttgccaaactggttcgcggtcacaaagaccagaaatggcgccggaggcgggaacaaggtggtggatgagtgctacatccccaattacttgctccccaaaacccagcctgagctccagtgggcgtggactaatatggaacagtatttaagcgcctgtttgaatctcacggagcgtaaacggttggtggcgcagcatctgacgcacgtgtcgcagacgcaggagcagaacaaagagaatcagaatcccaattctgatgcgccggtgatcagatcaaaaacttcagccaggtacatggagctggtcgggtggctcgtggacaaggggattacctcggagaagcagtggatccaggaggaccaggcctcatacatctccttcaatgcggcctccaactcgcggtcccaaatcaaggctgccttggacaatgcgggaaagattatgagcctgactaaaaccgcccccgactacctggtgggccagcagcccgtggaggacatttccagcaatcggatttataaaattttggaactaaacgggtacgatccccaatatgcggcttccgtctttctgggatgggccacgaaaaagttcggcaagaggaacaccatctggctgtttgggcctgcaactaccgggaagaccaacatcgcggaggccatagcccacactgtgcccttctacgggtgcgtaaactggaccaatgagaactttcccttcaacgactgtgtcgacaagatggtgatctggtgggaggaggggaagatgaccgccaaggtcgtggagtcggccaaagccattctcggaggaagcaaggtgcgcgtggaccagaaatgcaagtcctcggcccagatagacccgactcccgtgatcgtcacctccaacaccaacatgtgcgccgtgattgacgggaactcaacgaccttcgaacaccagcagccgttgcaagaccggatgttcaaatttgaactcacccgccgtctggatcatgactttgggaaggtcaccaagcaggaagtcaaagactttttccggtgggcaaaggatcacgtggttgaggtggagcatgaattctacgtcaaaaagggtggagccaagaaaagacccgcccccagtgacgcagatataagtgagcccaaacgggtgcgcgagtcagttgcgcagccatcgacgtcagacgcggaagcttcgatcaactacgcagacaggtaccaaaacaaatgttctcgtcacgtgggcatgaatctgatgctgtttccctgcagacaatgcgagagaatgaatcagaattcaaatatctgcttcactcacggacagaaagactgtttagagtgctttcccgtgtcagaatctcaacccgtttctgtcgtcaaaaaggcgtatcagaaactgtgctacattcatcatatcatgggaaaggtgccagacgcttgcactgcctgcgatctggtcaatgtggatttggatgactgcatctttgaacaataaatgatttaaatcaggtatggctgccgatggttatcttccagattggctcgaggacactctctctgaaggaataagacagtggtggaagctcaaacctggcccaccaccaccaaagcccgcagagcggcataaggacgacagcaggggtcttgtgcttcctgggtacaagtacctcggacccttcaacggactcgacaagggagagccggtcaacgaggcagacgccgcggccctcgagcacgacaaagcctacgaccggcagctcgacagcggagacaacccgtacctcaagtacaaccacgccgacgcggagtttcaggagcgccttaaagaagatacgtcttttgggggcaacctcggacgagcagtcttccaggcgaaaaagagggttcttgaacctctgggcctggttgaggaacctgttaagacggctccgggaaaaaagaggccggtagagcactctcctgtggagccagactcctcctcgggaaccggaaaggcgggccagcagcctgcaagaaaaagattgaattttggtcagactggagacgcagactcagtacctgacccccagcctctcggacagccaccagcagccccctctggtctgggaactaatacgatggctacaggcagtggcgcaccaatggcagacaataacgagggcgccgacggagtgggtaattcctcgggaaattggcattgcgattccacatggatgggcgacagagtcatcaccaccagcacccgaacctgggccctgcccacctacaacaaccacctctacaaacaaatttccagccaatcaggagcctcgaacgacaatcactactttggctacagcaccccttgggggtattttgacttcaacagattccactgccacttttcaccacgtgactggcaaagactcatcaacaacaactggggattccgacccaagagactcaacttcaagctctttaacattcaagtcaaagaggtcacgcagaatgacggtacgacgacgattgccaataaccttaccagcacggttcaggtgtttactgactcggagtaccagctcccgtacgtcctcggctcggcgcatcaaggatgcctcccgccgttcccagcagacgtcttcatggtgccacagtatggatacctcaccctgaacaacgggagtcaggcagtaggacgctcttcattttactgcctggagtactttccttctcagatgctgcgtaccggaaacaactttaccttcagctacacttttgaggacgttcctttccacagcagctacgctcacagccagagtctggaccgtctcatgaatcctctcatcgaccagtacctgtattacttgagcagaacaaacactccaagtggaaccaccacgcagtcaaggcttcagttttctcaggccggagcgagtgacattcgggaccagtctaggaactggcttcctggaccctgttaccgccagcagcgagtatcaaagacatctgcggataacaacaacagtgaatactcgtggactggagctaccaagtaccacctcaatggcagagactctctggtgaatccgggcccggccatggcaagccacaaggacgatgaagaaaagttttttcctcagagcggggttctcatctttgggaagcaaggctcagagaaaacaaatgtggacattgaaaaggtcatgattacagacgaagaggaaatcaggacaaccaatcccgtggctacggagcagtatggttctgtatctaccaacctccagcgcggccgcaacagacaagcagctaccgcagatgtcaacacacaaggcgttcttccaggcatggtctggcaggacagagatgtgtaccttcaggggcccatctgggcaaagattccacacacggacggacattttcacccctctcccctcatgggtggattcggacttaaacaccctcctccacagattctcatcaagaacaccccggtacctgcgaatccttcgaccaccttcagtgcggcaaagtttgcttccttcatcacacagtactccacgggacaggtcagcgtggagatcgagtgggagctgcagaaggaaaacagcaaacgctggaatcccgaaattcagtacacttccaactacaacaagtctgttaatgtggactttactgtggacactaatggcgtgtattcagagcctcgccccattggcaccagatacctgactcgtaatctgtaattgcttgttaatcaataaaccgtttaattcgtttcagttgaactttggtctctgcgtatttctttcttatctagtttccatggctacgtagataagtagcatggcgggttaatcattaactacagcccgggcgtttaaacagcgggcggaggggtggagtcgtgacgtgaattacgtcatagggttagggaggtcctgtattagaggtcacgtgagtgttttgcgacattttgcgacaccatgtggtctcgctgggggggggggcccgagtgagcacgcagggtctccattttgaagcgggaggtttgaacgagcgctggcgcgctcactggccgtcgttttacaacgtcgtgactgggaaaaccctggcgttacccaacttaatcgccttgcagcacatccccctttcgccagctggcgtaatagcgaagaggcccgcaccgatcgcccttcccaacagttgcgcagcctgaatggcgaatggaaattgtaagcgttaatattttgttaaaattcgcgttaaatttttgttaaatcagctcatttttttaaccaataggccgaaatcggcaaaatcccttataaatcaaaagaatagaccgagatagggttgagtgttgttccagtttggaacaagagtccactattaagaacgtggactccaacgtcaaagggcgaaaaaccgtctatcagggcgatggcccactacgtgaaccatcaccctaatcaagttttttggggtcgaggtgccgtaaagcactaaatcggaaccctaaagggagcccccgatttagagcttgacggggaaagccggcgaacgtggcgagaaaggaagggaagaaagcgaaaggagcgggcgctagggcgctggcaagtgtagcggtcacgctgcgcgtaaccaccacacccgccgcgcttaatgcgccgctacagggcgcgtcaggtggcacttttcggggaaatgtgcgcggaacccctatttgtttatttttctaaatacattcaaatatgtatccgctcatgagacaataaccctgataaatgcttcaataatattgaaaaaggaagagtatgagtattcaacatttccgtgtcgcccttattcccttttttgcggcattttgccttcctgtttttgctcacccagaaacgctggtgaaagtaaaagatgctgaagatcagttgggtgcacgagtgggttacatcgaactggatctcaacagcggtaagatccttgagagttttcgccccgaagaacgttttccaatgatgagcacttttaaagttctgctatgtggcgcggtattatcccgtattgacgccgggcaagagcaactcggtcgccgcatacactattctcagaatgacttggttgagtactcaccagtcacagaaaagcatcttacggatggcatgacagtaagagaattatgcagtgctgccataaccatgagtgataacactgcggccaacttacttctgacaacgatcggaggaccgaaggagctaaccgcttttttgcacaacatgggggatcatgtaactcgccttgatcgttgggaaccggagctgaatgaagccataccaaacgacgagcgtgacaccacgatgcctgtagcaatggcaacaacgttgcgcaaactattaactggcgaactacttactctagcttcccggcaacaattaatagactggatggaggcggataaagttgcaggaccacttctgcgctcggcccttccggctggctggtttattgctgataaatctggagccggtgagcgtgggtctcgcggtatcattgcagcactggggccagatggtaagccctcccgtatcgtagttatctacacgacggggagtcaggcaactatggatgaacgaaatagacagatcgctgagataggtgcctcactgattaagcattggtaactgtcagaccaagtttactcatatatactttagattgatttaaaacttcatttttaatttaaaaggatctaggtgaagatcctttttgataatctcatgaccaaaatcccttaacgtgagttttcgttccactgagcgtcagaccccgtagaaaagatcaaaggatcttcttgagatcctttttttctgcgcgtaatctgctgcttgcaaacaaaaaaaccaccgctaccagcggtggtttgtttgccggatcaagagctaccaactctttttccgaaggtaactggcttcagcagagcgcagataccaaatactgttcttctagtgtagccgtagttaggccaccacttcaagaactctgtagcaccgcctacatacctcgctctgctaatcctgttaccagtggctgctgccagtggcgataagtcgtgtcttaccgggttggactcaagacgatagttaccggataaggcgcagcggtcgggctgaacggggggttcgtgcacacagcccagcttggagcgaacgacctacaccgaactgagatacctacagcgtgagctatgagaaagcgccacgcttcccgaagggagaaaggcggacaggtatccggtaagcggcagggtcggaacaggagagcgcacgagggagcttccagggggaaacgcctggtatctttatagtcctgtcgggtttcgccacctctgacttgagcgtcgatttttgtgatgctcgtcaggggggcggagcctatggaaaaacgccagcaacgcggcctttttacggttcctggccttttgctggccttttgctcacatgttctttcctgcgttatcccctgattctgtggataaccgtattaccgcctttgagtgagctgataccgctcgccgcagccgaacgaccgagcgcagcgagtcagtgagcgaggaagcggaagagcgcccaatacgcaaaccgcctctccccgcgcgttggccgattcattaatgcagctggcacgacaggtttcccgactggaaagcgggcagtgagcgcaacgcaattaatgtgagttagctcactcattaggcaccccaggctttacactttatgcttccggctcgtatgttgtgtggaattgtgagcggataacaatttcacacaggaaacagctatgaccatgattacgccaa

SEQ ID NO: 14 - DNA, 65 bp, synthetic construct
  source 1..65: mol_type = other DNA
ggctgctgcatgggcccgtccgtttcctgctgctgcgttgcctctctggaggttggtagatacag

SEQ ID NO: 15 - DNA, 65 bp, synthetic construct
  source 1..65: mol_type = other DNA
gcagcagcaggaaacggacgggcccatgcagcagccagacaagcagctaccgcagatgtcaacac

SEQ ID NO: 16 - protein, 747 aa, synthetic construct
MAADGYLPDWLEDTLSEGIRQWWKLKPGPPPPKPAERHKDDSRGLVLPGYKYLGPFNGLDKGEPVNEADAAALEHDKAYDRQLDSGDNPYLKYNHADAEFQERLKEDTSFGGNLGRAVFQAKKRVLEPLGLVEEPVKTAPGKKRPVEHSPVEPDSSSGTGKAGQQPARKRLNFGQTGDADSVPDPQPLGQPPAAPSGLGTNTMATGSGAPMADNNEGADGVGNSSGNWHCDSTWMGDRVITTSTRTWALPTYNNHLYKQISSQSGASNDNHYFGYSTPWGYFDFNRFHCHFSPRDWQRLINNNWGFRPKRLNFKLFNIQVKEVTQNDGTTTIANNLTSTVQVFTDSEYQLPYVLGSAHQGCLPPFPADVFMVPQYGYLTLNNGSQAVGRSSFYCLEYFPSQMLRTGNNFTFSYTFEDVPFHSSYAHSQSLDRLMNPLIDQYLYYLSRTNTPSGTTTQSRLQFSQAGASDIRDQSRNWLPGPCYRQQRVSKTSADNNNSEYSWTGATKYHLNGRDSLVNPGPAMASHKDDEEKFFPQSGVLIFGKQGSEKTNVDIEKVMITDEEEIRTTNPVATEQYGSVSTNLQRGNAAAGNGRAHAAARQAATADVNTQGVLPGMVWQDRDVYLQGPIWAKIPHTDGHFHPSPLMGGFGLKHPPPQILIKNTPVPANPSTTFSAAKFASFITQYSTGQVSVEIEWELQKENSKRWNPEIQYTSNYNKSVNVDFTVDTNGVYSEPRPIGTRYLTRNL

SEQ ID NO: 17 - DNA, 22 bp, synthetic construct
  source 1..22: mol_type = other DNA
gcttctacccctctgacattgc

SEQ ID NO: 18 - DNA, 23 bp, synthetic construct
  source 1..23: mol_type = other DNA
caggaagaatgagccatcagagt

SEQ ID NO: 19 - DNA, 30 bp, synthetic construct
  source 1..30: mol_type = other DNA
ccagcctgagaacaactacaagacaacccc

SEQ ID NO: 20 - DNA, 1377 bp, synthetic construct
  source 1..1377: mol_type = other DNA
atggtgtcatactgggatactggagtcttgctttgtgccctgctgtcctgcctcctcctgactggctccagctcgggctcagataccggtcgccccttcgtggagatgtactccgagatcccggaaattatccacatgactgaggggcgcgaacttgtgatcccctgccgggtcaccagcccgaacattactgtgactttgaagaagttccccctggacaccctgattccggatgggaagagaattatctgggattcacggaagggattcatcatcagcaacgcgacctacaaggaaattggcctcctcacttgcgaagccactgtgaacggacacttgtacaagaccaactacctgacccaccgccagaccaacaccatcatcgacgtcgtcctgtccccttcgcacgggatcgagctctcggtgggagagaagttggtgcttaactgcaccgcccggacggaactgaatgtgggaatcgacttcaactgggaatacccgtccagcaagcatcagcataagaagctggtgaaccgggacctcaagactcagtccggcagcgaaatgaagaagttcctgtcgaccctcactattgacggagtgaccagatccgaccagggcctctacacttgcgccgcttccagcggactcatgaccaagaagaacagcactttcgtgagggtgcatgagaaggacaagacccacacgtgtccgccgtgcccagccccagagctgctgggaggcccttccgtgttcctgtttccgcccaagccaaaggataccctgatgatctcaaggacccctgaggtcacatgcgtcgtggtggatgtgtcgcacgaggaccctgaagtcaaattcaattggtatgtggacggagtggaagtccacaacgcgaaaaccaagccgagagaagaacagtacaattccacctaccgggtggtgtcggtgctgactgtgctgcaccaggactggctcaacggaaaggagtacaagtgcaaggtgtccaacaaggctctgcccgcacctattgaaaagaccatctccaaggccaagggtcaacctcgcgagcctcaggtgtacactctgcctccaagccgggacgaactgactaagaaccaagtctctctgacctgtttggtgaagggcttctacccgtcagacatcgcagtggagtgggagtcaaacggtcagccggagaacaactacaaaacaaccccccccgtgctggactccgacggctccttcttcctgtactccaagcttaccgtggataagagccgctggcaacagggcaacgtgttttcctgctccgtcatgcacgaagccctgcacaaccattatacccagaagtccctgtcgctgtcccccgggaaatag

SEQ ID NO: 21 - protein, 458 aa, synthetic construct
MVSYWDTGVLLCALLSCLLLTGSSSGSDTGRPFVEMYSEIPEIIHMTEGRELVIPCRVTSPNITVTLKKFPLDTLIPDGKRIIWDSRKGFIISNATYKEIGLLTCEATVNGHLYKTNYLTHRQTNTIIDVVLSPSHGIELSVGEKLVLNCTARTELNVGIDFNWEYPSSKHQHKKLVNRDLKTQSGSEMKKFLSTLTIDGVTRSDQGLYTCAASSGLMTKKNSTFVRVHEKDKTHTCPPCPAPELLGGPSVFLFPPKPKDTLMISRTPEVTCVVVDVSHEDPEVKFNWYVDGVEVHNAKTKPREEQYNSTYRVVSVLTVLHQDWLNGKEYKCKVSNKALPAPIEKTISKAKGQPREPQVYTLPPSRDELTKNQVSLTCLVKGFYPSDIAVEWESNGQPENNYKTTPPVLDSDGSFFLYSKLTVDKSRWQQGNVFSCSVMHEALHNHYTQKSLSLSPGK

SEQ ID NO: 22 - DNA, 1377 bp, synthetic construct
  source 1..1377: mol_type = other DNA
atggtgtcatactgggatactggagtcttgctttgtgccctgctgtcctgcctcctcctgactggctccagctcgggctctgatacaggcagaccctttgtggaaatgtactctgagattcctgaaatcatccacatgacagagggcagagaactggtgatcccatgcagagtgaccagccctaacatcacagtgacactgaagaagttcccactggacaccctgatccctgatggaaaaagaatcatttgggacagcaggaagggctttatcatcagtaatgccacctacaaagagataggcctgctcacatgtgaagctacagtgaatggccacctgtataaaacaaactacctgacccatagacagaccaataccatcatagatgtggtgctgagccccagccatggaatagagctgtctgtgggggagaagctggtactgaactgcactgccagaactgagcttaatgtgggcatagacttcaattgggagtaccccagctccaagcaccaacacaagaagctggtcaacagggacctgaagacccagagtggctctgaaatgaaaaagtttctgagcaccctgacaatagatggtgttacaaggagtgatcagggcctgtacacctgtgcagcttctagtggcctgatgaccaaaaagaacagcacctttgtgagggtgcatgagaaggacaagacacatacctgccctccatgtcctgcccctgaactgctgggaggacctagtgtgtttctgttcccccccaagcctaaggacaccctgatgatcagcaggacccctgaggtgacatgtgtggtggtggatgtgtctcatgaggacccagaggtgaagttcaactggtatgtggatggggtggaagtgcacaatgccaaaaccaagcccagagaggaacagtacaacagcacatacagggtggtgtctgtgctgacagtcctgcaccaggattggctgaatggaaaggaatacaagtgcaaggtgtccaacaaggccctgcctgctcctatagagaagaccatcagcaaggccaagggccagcctagagagcctcaggtgtacaccctgcctccctccagagatgagctgacaaagaaccaggtgtccctgacttgcctggtcaagggcttctaccctagtgacatagcagtggaatgggaaagcaatggccaacctgagaacaactacaagacaacccccccagtgttggattcagatggcagcttcttcctgtacagcaagctgacagtggacaaaagcaggtggcagcagggcaatgtgttcagctgcagtgtgatgcatgaggccctgcacaatcactacacacagaaaagcctgagcctgtctcctggcaaatga

SEQ ID NO: 23 - DNA, 1377 bp, synthetic construct
  source 1..1377: mol_type = other DNA
atggtgtcatactgggatactggagtcttgctttgtgccctgctgtcctgcctcctcctgactggctccagctcgggctctgacacaggcagaccctttgtggaaatgtactctgagatccctgagatcatccacatgacagagggcagagagctggtcatcccctgcagagtgacaagccccaacatcacagtgaccctgaagaagttccctctggacacactgatccctgatggcaagagaatcatctgggacagcagaaagggcttcatcatcagcaatgccacctacaaagagattggcctgctgacctgtgaagccacagtgaatggccacctgtacaagaccaactacctgacacacagacagaccaacaccatcattgatgtggtgctgagccccagccatggcattgagctgtctgtgggagagaagctggtgctgaactgcacagccagaacagagctgaatgtgggcattgacttcaactgggagtaccccagcagcaagcaccagcacaagaaactggtcaacagggacctgaaaacccagagtggctctgagatgaagaaattcctgagcaccctgaccattgatggggtcaccagatctgaccagggcctgtacacatgtgctgccagctctggactgatgaccaagaaaaacagcacctttgtcagagtgcatgagaaggacaagacccacacctgtcctccatgtcctgcacctgagctgcttggaggcccctctgtgttcctgtttcctccaaagcctaaggacaccctgatgatcagcagaacacctgaagtgacctgtgtggtggtggatgtgtcccatgaggacccagaagtgaagttcaattggtatgtggatggggttgaagtgcacaatgccaagaccaagcctagagaggaacagtacaactccacctacagagtggtgtcagtgctgacagtgctgcaccaggactggctgaatggcaaagagtacaagtgcaaggtgtccaacaaggccctgcctgctcctattgagaaaaccatctccaaggccaagggccagcctagggaaccccaggtttacacactgccacctagcagggatgagctgacaaagaaccaggtgtccctgacctgcctggtcaagggcttctacccctctgacattgctgtggaatgggagagcaatggccagcctgagaacaactacaagacaacccctcctgtgctggactctgatggctcattcttcctgtacagcaagctgactgtggacaagagcagatggcagcagggaaatgtgttcagctgctctgtgatgcatgaggccctgcacaaccactacacccagaaaagcctgagcctgtctcctggcaagtga

SEQ ID NO: 24 - DNA, 3050 bp, synthetic construct
  source 1..3050: mol_type = other DNA
acgcgtctagttattaatagtaatcaattacggggtcattagttcatagcccatatatggagttccgcgttacataacttacggtaaatggcccgcctggctgaccgcccaacgacccccgcccattgacgtcaataatgacgtatgttcccatagtaacgccaatagggactttccattgacgtcaatgggtggagtatttacggtaaactgcccacttggcagtacatcaagtgtatcatatgccaagtacgccccctattgacgtcaatgacggtaaatggcccgcctggcattatgcccagtacatgaccttatgggactttcctacttggcagtacatctacgtattagtcatcgctattaccatggtgatgcggttttggcagtacatcaatgggcgtggatagcggtttgactcacggggatttccaagtctccaccccattgacgtcaatgggagtttgttttggcaccaaaatcaacgggactttccaaaatgtcgtaacaactccgccccattgacgcaaatgggcggtaggcgtgtacggtgggaggtctatataagcagagctcgtttagtgaaccgtcagatcgcctggagacgccatccacgctgttttgacctccatagaagacaccgggaccgatccagcctccgcggattcgaatcccggccgggaacggtgcattggaacgcggattccccgtgccaagagtgacgtaagtaccgcctatagagtctataggcccacaaaaaatgctttcttcttttaatatacttttttgtttatcttatttctaatactttccctaatctctttctttcagggcaataatgatacaatgtatcatgcctctttgcaccattctaaagaataacagtgataatttctgggttaaggcaatagcaatatttctgcatataaatatttctgcatataaattgtaactgatgtaagaggtttcatattgctaatagcagctacaatccagctaccattctgcttttattttatggttgggataaggctggattattctgagtccaagctaggcccttttgctaatcatgttcatacctcttatcttcctcccacagctcctgggcaacgtgctggtctgtgtgctggcccatcactttggcaaagaattgggataattactagatcgccaccatggtgtcatactgggatactggagtcttgctttgtgccctgctgtcctgcctcctcctgactggctccagctcgggctcagataccggtcgccccttcgtggagatgtactccgagatcccggaaattatccacatgactgaggggcgcgaacttgtgatcccctgccgggtcaccagcccgaacattactgtgactttgaagaagttccccctggacaccctgattccggatgggaagagaattatctgggattcacggaagggattcatcatcagcaacgcgacctacaaggaaattggcctcctcacttgcgaagccactgtgaacggacacttgtacaagaccaactacctgacccaccgccagaccaacaccatcatcgacgtcgtcctgtccccttcgcacgggatcgagctctcggtgggagagaagttggtgcttaactgcaccgcccggacggaactgaatgtgggaatcgacttcaactgggaatacccgtccagcaagcatcagcataagaagctggtgaaccgggacctcaagactcagtccggcagcgaaatgaagaagttcctgtcgaccctcactattgacggagtgaccagatccgaccagggcctctacacttgcgccgcttccagcggactcatgaccaagaagaacagcactttcgtgagggtgcatgagaaggacaagacccacacgtgtccgccgtgcccagccccagagctgctgggaggcccttccgtgttcctgtttccgcccaagccaaaggataccctgatgatctcaaggacccctgaggtcacatgcgtcgtggtggatgtgtcgcacgaggaccctgaagtcaaattcaattggtatgtggacggagtggaagtccacaacgcgaaaaccaagccgagagaagaacagtacaattccacctaccgggtggtgtcggtgctgactgtgctgcaccaggactggctcaacggaaaggagtacaagtgcaaggtgtccaacaaggctctgcccgcacctattgaaaagaccatctccaaggccaagggtcaacctcgcgagcctcaggtgtacactctgcctccaagccgggacgaactgactaagaaccaagtctctctgacctgtttggtgaagggcttctacccgtcagacatcgcagtggagtgggagtcaaacggtcagccggagaacaactacaaaacaaccccccccgtgctggactccgacggctccttcttcctgtactccaagcttaccgtggataagagccgctggcaacagggcaacgtgttttcctgctccgtcatgcacgaagccctgcacaaccattatacccagaagtccctgtcgctgtcccccgggaaataggcggccgcaagcttcgggtggcatccctgtgacccctccccagtgcctctcctggccctggaagttgccactccagtgcccaccagccttgtcctaataaaattaagttgcatcattttgtctgactaggtgtccttctataatattatggggtggaggggggtggtatggagcaaggggcaagttgggaagacaacctgtagggcctgcggggtctattgggaaccaagctggagtgcagtggcacaatcttggctcactgcaatctccgcctcctgggttcaagcgattctcctgcctcagcctcccgagttgttgggattccaggcatgcatgaccaggctcagctaatttttgtttttttggtagagacggggtttcaccatattggccaggctggtctccaactcctaatctcaggtgatctacccaccttggcctcccaaattgctgggattacaggcgtgaaccactgctcccttccctgtccttcgg

SEQ ID NO: 25 - DNA, 54 bp, synthetic construct
  source 1..54: mol_type = other DNA
atgaagtgggtgaccttcatcagcctgctgttcctgttttcttcagcctacagc

SEQ ID NO: 26 - DNA, 57 bp, synthetic construct
  source 1..57: mol_type = other DNA
atgagactgctggccttcctgagcctgctggccctggtgctgcaggagacaggcacc

SEQ ID NO: 27 - DNA, 60 bp, synthetic construct
  source 1..60: mol_type = other DNA
atgtacagaatgcagctgctgagctgcatagccctgtctctggccctggtgaccaacagc

SEQ ID NO: 28 - DNA, 87 bp, synthetic construct
  source 1..87: mol_type = other DNA
atgcacagacccagaaggaggggcaccagacctccacctctggctctgctggcagccctgctgctggcagctagaggagcagatgcc

SEQ ID NO: 29 - DNA, 1353 bp, synthetic construct
  source 1..1353: mol_type = other DNA
atgaagtgggtgaccttcatcagcctgctgttcctgttttcttcagcctacagctctgacacaggcagaccctttgtggaaatgtactctgagatccctgagatcatccacatgacagagggcagagagctggtcatcccctgcagagtgacaagccccaacatcacagtgaccctgaagaagttccctctggacacactgatccctgatggcaagagaatcatctgggacagcagaaagggcttcatcatcagcaatgccacctacaaagagattggcctgctgacctgtgaagccacagtgaatggccacctgtacaagaccaactacctgacacacagacagaccaacaccatcattgatgtggtgctgagccccagccatggcattgagctgtctgtgggagagaagctggtgctgaactgcacagccagaacagagctgaatgtgggcattgacttcaactgggagtaccccagcagcaagcaccagcacaagaaactggtcaacagggacctgaaaacccagagtggctctgagatgaagaaattcctgagcaccctgaccattgatggggtcaccagatctgaccagggcctgtacacatgtgctgccagctctggactgatgaccaagaaaaacagcacctttgtcagagtgcatgagaaggacaagacccacacctgtcctccatgtcctgcacctgagctgcttggaggcccctctgtgttcctgtttcctccaaagcctaaggacaccctgatgatcagcagaacacctgaagtgacctgtgtggtggtggatgtgtcccatgaggacccagaagtgaagttcaattggtatgtggatggggttgaagtgcacaatgccaagaccaagcctagagaggaacagtacaactccacctacagagtggtgtcagtgctgacagtgctgcaccaggactggctgaatggcaaagagtacaagtgcaaggtgtccaacaaggccctgcctgctcctattgagaaaaccatctccaaggccaagggccagcctagggaaccccaggtttacacactgccacctagcagggatgagctgacaaagaaccaggtgtccctgacctgcctggtcaagggcttctacccctctgacattgctgtggaatgggagagcaatggccagcctgagaacaactacaagacaacccctcctgtgctggactctgatggctcattcttcctgtacagcaagctgactgtggacaagagcagatggcagcagggaaatgtgttcagctgctctgtgatgcatgaggccctgcacaaccactacacccagaaaagcctgagcctgtctcctggcaagtga

SEQ ID NO: 30 - protein, 450 aa, synthetic construct
MKWVTFISLLFLFSSAYSSDTGRPFVEMYSEIPEIIHMTEGRELVIPCRVTSPNITVTLKKFPLDTLIPDGKRIIWDSRKGFIISNATYKEIGLLTCEATVNGHLYKTNYLTHRQTNTIIDVVLSPSHGIELSVGEKLVLNCTARTELNVGIDFNWEYPSSKHQHKKLVNRDLKTQSGSEMKKFLSTLTIDGVTRSDQGLYTCAASSGLMTKKNSTFVRVHEKDKTHTCPPCPAPELLGGPSVFLFPPKPKDTLMISRTPEVTCVVVDVSHEDPEVKFNWYVDGVEVHNAKTKPREEQYNSTYRVVSVLTVLHQDWLNGKEYKCKVSNKALPAPIEKTISKAKGQPREPQVYTLPPSRDELTKNQVSLTCLVKGFYPSDIAVEWESNGQPENNYKTTPPVLDSDGSFFLYSKLTVDKSRWQQGNVFSCSVMHEALHNHYTQKSLSLSPGK

SEQ ID NO: 31 - DNA, 1356 bp, synthetic construct
  source 1..1356: mol_type = other DNA
atgagactgctggccttcctgagcctgctggccctggtgctgcaggagacaggcacctctgacacaggcagaccctttgtggaaatgtactctgagatccctgagatcatccacatgacagagggcagagagctggtcatcccctgcagagtgacaagccccaacatcacagtgaccctgaagaagttccctctggacacactgatccctgatggcaagagaatcatctgggacagcagaaagggcttcatcatcagcaatgccacctacaaagagattggcctgctgacctgtgaagccacagtgaatggccacctgtacaagaccaactacctgacacacagacagaccaacaccatcattgatgtggtgctgagccccagccatggcattgagctgtctgtgggagagaagctggtgctgaactgcacagccagaacagagctgaatgtgggcattgacttcaactgggagtaccccagcagcaagcaccagcacaagaaactggtcaacagggacctgaaaacccagagtggctctgagatgaagaaattcctgagcaccctgaccattgatggggtcaccagatctgaccagggcctgtacacatgtgctgccagctctggactgatgaccaagaaaaacagcacctttgtcagagtgcatgagaaggacaagacccacacctgtcctccatgtcctgcacctgagctgcttggaggcccctctgtgttcctgtttcctccaaagcctaaggacaccctgatgatcagcagaacacctgaagtgacctgtgtggtggtggatgtgtcccatgaggacccagaagtgaagttcaattggtatgtggatggggttgaagtgcacaatgccaagaccaagcctagagaggaacagtacaactccacctacagagtggtgtcagtgctgacagtgctgcaccaggactggctgaatggcaaagagtacaagtgcaaggtgtccaacaaggccctgcctgctcctattgagaaaaccatctccaaggccaagggccagcctagggaaccccaggtttacacactgccacctagcagggatgagctgacaaagaaccaggtgtccctgacctgcctggtcaagggcttctacccctctgacattgctgtggaatgggagagcaatggccagcctgagaacaactacaagacaacccctcctgtgctggactctgatggctcattcttcctgtacagcaagctgactgtggacaagagcagatggcagcagggaaatgtgttcagctgctctgtgatgcatgaggccctgcacaaccactacacccagaaaagcctgagcctgtctcctggcaagtga

SEQ ID NO: 32 - protein, 451 aa, synthetic construct
MRLLAFLSLLALVLQETGTSDTGRPFVEMYSEIPEIIHMTEGRELVIPCRVTSPNITVTLKKFPLDTLIPDGKRIIWDSRKGFIISNATYKEIGLLTCEATVNGHLYKTNYLTHRQTNTIIDVVLSPSHGIELSVGEKLVLNCTARTELNVGIDFNWEYPSSKHQHKKLVNRDLKTQSGSEMKKFLSTLTIDGVTRSDQGLYTCAASSGLMTKKNSTFVRVHEKDKTHTCPPCPAPELLGGPSVFLFPPKPKDTLMISRTPEVTCVVVDVSHEDPEVKFNWYVDGVEVHNAKTKPREEQYNSTYRVVSVLTVLHQDWLNGKEYKCKVSNKALPAPIEKTISKAKGQPREPQVYTLPPSRDELTKNQVSLTCLVKGFYPSDIAVEWESNGQPENNYKTTPPVLDSDGSFFLYSKLTVDKSRWQQGNVFSCSVMHEALHNHYTQKSLSLSPGK

SEQ ID NO: 33 - DNA, 1386 bp, synthetic construct
  source 1..1386: mol_type = other DNA
atgcacagacccagaaggaggggcaccagacctccacctctggctctgctggcagccctgctgctggcagctagaggagcagatgcctctgacacaggcagaccctttgtggaaatgtactctgagatccctgagatcatccacatgacagagggcagagagctggtcatcccctgcagagtgacaagccccaacatcacagtgaccctgaagaagttccctctggacacactgatccctgatggcaagagaatcatctgggacagcagaaagggcttcatcatcagcaatgccacctacaaagagattggcctgctgacctgtgaagccacagtgaatggccacctgtacaagaccaactacctgacacacagacagaccaacaccatcattgatgtggtgctgagccccagccatggcattgagctgtctgtgggagagaagctggtgctgaactgcacagccagaacagagctgaatgtgggcattgacttcaactgggagtaccccagcagcaagcaccagcacaagaaactggtcaacagggacctgaaaacccagagtggctctgagatgaagaaattcctgagcaccctgaccattgatggggtcaccagatctgaccagggcctgtacacatgtgctgccagctctggactgatgaccaagaaaaacagcacctttgtcagagtgcatgagaaggacaagacccacacctgtcctccatgtcctgcacctgagctgcttggaggcccctctgtgttcctgtttcctccaaagcctaaggacaccctgatgatcagcagaacacctgaagtgacctgtgtggtggtggatgtgtcccatgaggacccagaagtgaagttcaattggtatgtggatggggttgaagtgcacaatgccaagaccaagcctagagaggaacagtacaactccacctacagagtggtgtcagtgctgacagtgctgcaccaggactggctgaatggcaaagagtacaagtgcaaggtgtccaacaaggccctgcctgctcctattgagaaaaccatctccaaggccaagggccagcctagggaaccccaggtttacacactgccacctagcagggatgagctgacaaagaaccaggtgtccctgacctgcctggtcaagggcttctacccctctgacattgctgtggaatgggagagcaatggccagcctgagaacaactacaagacaacccctcctgtgctggactctgatggctcattcttcctgtacagcaagctgactgtggacaagagcagatggcagcagggaaatgtgttcagctgctctgtgatgcatgaggccctgcacaaccactacacccagaaaagcctgagcctgtctcctggcaagtga

SEQ ID NO: 34 - protein, 461 aa, synthetic construct
MHRPRRRGTRPPPLALLAALLLAARGADASDTGRPFVEMYSEIPEIIHMTEGRELVIPCRVTSPNITVTLKKFPLDTLIPDGKRIIWDSRKGFIISNATYKEIGLLTCEATVNGHLYKTNYLTHRQTNTIIDVVLSPSHGIELSVGEKLVLNCTARTELNVGIDFNWEYPSSKHQHKKLVNRDLKTQSGSEMKKFLSTLTIDGVTRSDQGLYTCAASSGLMTKKNSTFVRVHEKDKTHTCPPCPAPELLGGPSVFLFPPKPKDTLMISRTPEVTCVVVDVSHEDPEVKFNWYVDGVEVHNAKTKPREEQYNSTYRVVSVLTVLHQDWLNGKEYKCKVSNKALPAPIEKTISKAKGQPREPQVYTLPPSRDELTKNQVSLTCLVKGFYPSDIAVEWESNGQPENNYKTTPPVLDSDGSFFLYSKLTVDKSRWQQGNVFSCSVMHEALHNHYTQKSLSLSPGK

SEQ ID NO: 35 - DNA, 3026 bp, synthetic construct
  source 1..3026: mol_type = other DNA
acgcgtctagttattaatagtaatcaattacggggtcattagttcatagcccatatatggagttccgcgttacataacttacggtaaatggcccgcctggctgaccgcccaacgacccccgcccattgacgtcaataatgacgtatgttcccatagtaacgccaatagggactttccattgacgtcaatgggtggagtatttacggtaaactgcccacttggcagtacatcaagtgtatcatatgccaagtacgccccctattgacgtcaatgacggtaaatggcccgcctggcattatgcccagtacatgaccttatgggactttcctacttggcagtacatctacgtattagtcatcgctattaccatggtgatgcggttttggcagtacatcaatgggcgtggatagcggtttgactcacggggatttccaagtctccaccccattgacgtcaatgggagtttgttttggcaccaaaatcaacgggactttccaaaatgtcgtaacaactccgccccattgacgcaaatgggcggtaggcgtgtacggtgggaggtctatataagcagagctcgtttagtgaaccgtcagatcgcctggagacgccatccacgctgttttgacctccatagaagacaccgggaccgatccagcctccgcggattcgaatcccggccgggaacggtgcattggaacgcggattccccgtgccaagagtgacgtaagtaccgcctatagagtctataggcccacaaaaaatgctttcttcttttaatatacttttttgtttatcttatttctaatactttccctaatctctttctttcagggcaataatgatacaatgtatcatgcctctttgcaccattctaaagaataacagtgataatttctgggttaaggcaatagcaatatttctgcatataaatatttctgcatataaattgtaactgatgtaagaggtttcatattgctaatagcagctacaatccagctaccattctgcttttattttatggttgggataaggctggattattctgagtccaagctaggcccttttgctaatcatgttcatacctcttatcttcctcccacagctcctgggcaacgtgctggtctgtgtgctggcccatcactttggcaaagaattgggataattactagatcgccaccatgaagtgggtgaccttcatcagcctgctgttcctgttttcttcagcctacagctctgacacaggcagaccctttgtggaaatgtactctgagatccctgagatcatccacatgacagagggcagagagctggtcatcccctgcagagtgacaagccccaacatcacagtgaccctgaagaagttccctctggacacactgatccctgatggcaagagaatcatctgggacagcagaaagggcttcatcatcagcaatgccacctacaaagagattggcctgctgacctgtgaagccacagtgaatggccacctgtacaagaccaactacctgacacacagacagaccaacaccatcattgatgtggtgctgagccccagccatggcattgagctgtctgtgggagagaagctggtgctgaactgcacagccagaacagagctgaatgtgggcattgacttcaactgggagtaccccagcagcaagcaccagcacaagaaactggtcaacagggacctgaaaacccagagtggctctgagatgaagaaattcctgagcaccctgaccattgatggggtcaccagatctgaccagggcctgtacacatgtgctgccagctctggactgatgaccaagaaaaacagcacctttgtcagagtgcatgagaaggacaagacccacacctgtcctccatgtcctgcacctgagctgcttggaggcccctctgtgttcctgtttcctccaaagcctaaggacaccctgatgatcagcagaacacctgaagtgacctgtgtggtggtggatgtgtcccatgaggacccagaagtgaagttcaattggtatgtggatggggttgaagtgcacaatgccaagaccaagcctagagaggaacagtacaactccacctacagagtggtgtcagtgctgacagtgctgcaccaggactggctgaatggcaaagagtacaagtgcaaggtgtccaacaaggccctgcctgctcctattgagaaaaccatctccaaggccaagggccagcctagggaaccccaggtttacacactgccacctagcagggatgagctgacaaagaaccaggtgtccctgacctgcctggtcaagggcttctacccctctgacattgctgtggaatgggagagcaatggccagcctgagaacaactacaagacaacccctcctgtgctggactctgatggctcattcttcctgtacagcaagctgactgtggacaagagcagatggcagcagggaaatgtgttcagctgctctgtgatgcatgaggccctgcacaaccactacacccagaaaagcctgagcctgtctcctggcaagtgagcggccgcaagcttcgggtggcatccctgtgacccctccccagtgcctctcctggccctggaagttgccactccagtgcccaccagccttgtcctaataaaattaagttgcatcattttgtctgactaggtgtccttctataatattatggggtggaggggggtggtatggagcaaggggcaagttgggaagacaacctgtagggcctgcggggtctattgggaaccaagctggagtgcagtggcacaatcttggctcactgcaatctccgcctcctgggttcaagcgattctcctgcctcagcctcccgagttgttgggattccaggcatgcatgaccaggctcagctaatttttgtttttttggtagagacggggtttcaccatattggccaggctggtctccaactcctaatctcaggtgatctacccaccttggcctcccaaattgctgggattacaggcgtgaaccactgctcccttccctgtccttcgg

SEQ ID NO: 36 - DNA, 2740 bp, synthetic construct
  source 1..2740: mol_type = other DNA
acgcgtctagttattaatagtaatcaattacggggtcattagttcatagcccatatatggagttccgcgttacataacttacggtaaatggcccgcctggctgaccgcccaacgacccccgcccattgacgtcaataatgacgtatgttcccatagtaacgccaatagggactttccattgacgtcaatgggtggagtatttacggtaaactgcccacttggcagtacatcaagtgtatcatatgccaagtacgccccctattgacgtcaatgacggtaaatggcccgcctggcattatgcccagtacatgaccttacgggactttcctacttggcagtacatctacgtattagtcatcgctattaccatggtcgaggtgagccccacgttctgcttcactctccccatctcccccccctccccacccccaattttgtatttatttattttttaattattttgtgcagcgatgggggcggggggggggggggcgcgcgccaggcggggcggggcggggcgaggggcggggcggggcgaggcggagaggtgcggcggcagccaatcagagcggcgcgctccgaaagtttccttttatggcgaggcggcggcggcggcggccctataaaaagcgaagcgcgcggcgggcggggagtcgctgcgttgccttcgccccgtgccccgctccgcgccgcctcgcgccgcccgccccggctctgactgaccgcgttactcccacaggtgagcgggcgggacggcccttctcctccgggctgtaattagcaagaggtaagggtttaagggatggttggttggtggggtattaatgtttaattacctgttttacaggcctgaaatcacttggttttaggttggaattactagatcgccaccatgaagtgggtgaccttcatcagcctgctgttcctgttttcttcagcctacagctctgacacaggcagaccctttgtggaaatgtactctgagatccctgagatcatccacatgacagagggcagagagctggtcatcccctgcagagtgacaagccccaacatcacagtgaccctgaagaagttccctctggacacactgatccctgatggcaagagaatcatctgggacagcagaaagggcttcatcatcagcaatgccacctacaaagagattggcctgctgacctgtgaagccacagtgaatggccacctgtacaagaccaactacctgacacacagacagaccaacaccatcattgatgtggtgctgagccccagccatggcattgagctgtctgtgggagagaagctggtgctgaactgcacagccagaacagagctgaatgtgggcattgacttcaactgggagtaccccagcagcaagcaccagcacaagaaactggtcaacagggacctgaaaacccagagtggctctgagatgaagaaattcctgagcaccctgaccattgatggggtcaccagatctgaccagggcctgtacacatgtgctgccagctctggactgatgaccaagaaaaacagcacctttgtcagagtgcatgagaaggacaagacccacacctgtcctccatgtcctgcacctgagctgcttggaggcccctctgtgttcctgtttcctccaaagcctaaggacaccctgatgatcagcagaacacctgaagtgacctgtgtggtggtggatgtgtcccatgaggacccagaagtgaagttcaattggtatgtggatggggttgaagtgcacaatgccaagaccaagcctagagaggaacagtacaactccacctacagagtggtgtcagtgctgacagtgctgcaccaggactggctgaatggcaaagagtacaagtgcaaggtgtccaacaaggccctgcctgctcctattgagaaaaccatctccaaggccaagggccagcctagggaaccccaggtttacacactgccacctagcagggatgagctgacaaagaaccaggtgtccctgacctgcctggtcaagggcttctacccctctgacattgctgtggaatgggagagcaatggccagcctgagaacaactacaagacaacccctcctgtgctggactctgatggctcattcttcctgtacagcaagctgactgtggacaagagcagatggcagcagggaaatgtgttcagctgctctgtgatgcatgaggccctgcacaaccactacacccagaaaagcctgagcctgtctcctggcaagtgagcggccgcaagcttcgggtggcatccctgtgacccctccccagtgcctctcctggccctggaagttgccactccagtgcccaccagccttgtcctaataaaattaagttgcatcattttgtctgactaggtgtccttctataatattatggggtggaggggggtggtatggagcaaggggcaagttgggaagacaacctgtagggcctgcggggtctattgggaaccaagctggagtgcagtggcacaatcttggctcactgcaatctccgcctcctgggttcaagcgattctcctgcctcagcctcccgagttgttgggattccaggcatgcatgaccaggctcagctaatttttgtttttttggtagagacggggtttcaccatattggccaggctggtctccaactcctaatctcaggtgatctacccaccttggcctcccaaattgctgggattacaggcgtgaaccactgctcccttccctgtccttcgg

SEQ ID NO: 37 - DNA, 3580 bp, synthetic construct
  source 1..3580: mol_type = other DNA
acgcgtctagttattaatagtaatcaattacggggtcattagttcatagcccatatatggagttccgcgttacataacttacggtaaatggcccgcctggctgaccgcccaacgacccccgcccattgacgtcaataatgacgtatgttcccatagtaacgccaatagggactttccattgacgtcaatgggtggagtatttacggtaaactgcccacttggcagtacatcaagtgtatcatatgccaagtacgccccctattgacgtcaatgacggtaaatggcccgcctggcattatgcccagtacatgaccttacgggactttcctacttggcagtacatctacgtattagtcatcgctattaccatggtcgaggtgagccccacgttctgcttcactctccccatctcccccccctccccacccccaattttgtatttatttattttttaattattttgtgcagcgatgggggcggggggggggggggcgcgcgccaggcggggcggggcggggcgaggggcggggcggggcgaggcggagaggtgcggcggcagccaatcagagcggcgcgctccgaaagtttccttttatggcgaggcggcggcggcggcggccctataaaaagcgaagcgcgcggcgggcgggagtcgctgcgcgctgccttcgccccgtgccccgctccgccgccgcctcgcgccgcccgccccggctctgactgaccgcgttactcccacaggtgagcgggcgggacggcccttctcctccgggctgtaattagcgcttggtttaatgacggcttgtttcttttctgtggctgcgtgaaagccttgaggggctccgggagggccctttgtgcggggggagcggctcggggggtgcgtgcgtgtgtgtgtgcgtggggagcgccgcgtgcggctccgcgctgcccggcggctgtgagcgctgcgggcgcggcgcggggctttgtgcgctccgcagtgtgcgcgaggggagcgcggccgggggcggtgccccgcggtgcggggggggctgcgaggggaacaaaggctgcgtgcggggtgtgtgcgtgggggggtgagcagggggtgtgggcgcgtcggtcgggctgcaaccccccctgcacccccctccccgagttgctgagcacggcccggcttcgggtgcggggctccgtacggggcgtggcgcggggctcgccgtgccgggcggggggtggcggcaggtgggggtgccgggcggggcggggccgcctcgggccggggagggctcgggggaggggcgcggcggcccccggagcgccggcggctgtcgaggcgcggcgagccgcagccattgccttttatggtaatcgtgcgagagggcgcagggacttcctttgtcccaaatctgtgcggagccgaaatctgggaggcgccgccgcaccccctctagcgggcgcggggcgaagcggtgcggcgccggcaggaaggaaatgggcggggagggccttcgtgcgtcgccgcgccgccgtccccttctccctctccagcctcggggctgtccgcggggggacggctgccttcgggggggacggggcagggcggggttcggcttctggcgtgtgaccggcggctctagagcctctgctaaccatgttcatgccttcttctttttcctacagctcctgggcaacgtgctggttattgtgctgtctcatcattttggcaaagaattactagatcgccaccatgaagtgggtgaccttcatcagcctgctgttcctgttttcttcagcctacagctctgacacaggcagaccctttgtggaaatgtactctgagatccctgagatcatccacatgacagagggcagagagctggtcatcccctgcagagtgacaagccccaacatcacagtgaccctgaagaagttccctctggacacactgatccctgatggcaagagaatcatctgggacagcagaaagggcttcatcatcagcaatgccacctacaaagagattggcctgctgacctgtgaagccacagtgaatggccacctgtacaagaccaactacctgacacacagacagaccaacaccatcattgatgtggtgctgagccccagccatggcattgagctgtctgtgggagagaagctggtgctgaactgcacagccagaacagagctgaatgtgggcattgacttcaactgggagtaccccagcagcaagcaccagcacaagaaactggtcaacagggacctgaaaacccagagtggctctgagatgaagaaattcctgagcaccctgaccattgatggggtcaccagatctgaccagggcctgtacacatgtgctgccagctctggactgatgaccaagaaaaacagcacctttgtcagagtgcatgagaaggacaagacccacacctgtcctccatgtcctgcacctgagctgcttggaggcccctctgtgttcctgtttcctccaaagcctaaggacaccctgatgatcagcagaacacctgaagtgacctgtgtggtggtggatgtgtcccatgaggacccagaagtgaagttcaattggtatgtggatggggttgaagtgcacaatgccaagaccaagcctagagaggaacagtacaactccacctacagagtggtgtcagtgctgacagtgctgcaccaggactggctgaatggcaaagagtacaagtgcaaggtgtccaacaaggccctgcctgctcctattgagaaaaccatctccaaggccaagggccagcctagggaaccccaggtttacacactgccacctagcagggatgagctgacaaagaaccaggtgtccctgacctgcctggtcaagggcttctacccctctgacattgctgtggaatgggagagcaatggccagcctgagaacaactacaagacaacccctcctgtgctggactctgatggctcattcttcctgtacagcaagctgactgtggacaagagcagatggcagcagggaaatgtgttcagctgctctgtgatgcatgaggccctgcacaaccactacacccagaaaagcctgagcctgtctcctggcaagtgagcggccgcaagcttcgggtggcatccctgtgacccctccccagtgcctctcctggccctggaagttgccactccagtgcccaccagccttgtcctaataaaattaagttgcatcattttgtctgactaggtgtccttctataatattatggggtggaggggggtggtatggagcaaggggcaagttgggaagacaacctgtagggcctgcggggtctattgggaaccaagctggagtgcagtggcacaatcttggctcactgcaatctccgcctcctgggttcaagcgattctcctgcctcagcctcccgagttgttgggattccaggcatgcatgaccaggctcagctaatttttgtttttttggtagagacggggtttcaccatattggccaggctggtctccaactcctaatctcaggtgatctacccaccttggcctcccaaattgctgggattacaggcgtgaaccactgctcccttccctgtccttcgg

SEQ ID NO: 38 - DNA, 3029 bp, synthetic construct
  source 1..3029: mol_type = other DNA
acgcgtctagttattaatagtaatcaattacggggtcattagttcatagcccatatatggagttccgcgttacataacttacggtaaatggcccgcctggctgaccgcccaacgacccccgcccattgacgtcaataatgacgtatgttcccatagtaacgccaatagggactttccattgacgtcaatgggtggagtatttacggtaaactgcccacttggcagtacatcaagtgtatcatatgccaagtacgccccctattgacgtcaatgacggtaaatggcccgcctggcattatgcccagtacatgaccttatgggactttcctacttggcagtacatctacgtattagtcatcgctattaccatggtgatgcggttttggcagtacatcaatgggcgtggatagcggtttgactcacggggatttccaagtctccaccccattgacgtcaatgggagtttgttttggcaccaaaatcaacgggactttccaaaatgtcgtaacaactccgccccattgacgcaaatgggcggtaggcgtgtacggtgggaggtctatataagcagagctcgtttagtgaaccgtcagatcgcctggagacgccatccacgctgttttgacctccatagaagacaccgggaccgatccagcctccgcggattcgaatcccggccgggaacggtgcattggaacgcggattccccgtgccaagagtgacgtaagtaccgcctatagagtctataggcccacaaaaaatgctttcttcttttaatatacttttttgtttatcttatttctaatactttccctaatctctttctttcagggcaataatgatacaatgtatcatgcctctttgcaccattctaaagaataacagtgataatttctgggttaaggcaatagcaatatttctgcatataaatatttctgcatataaattgtaactgatgtaagaggtttcatattgctaatagcagctacaatccagctaccattctgcttttattttatggttgggataaggctggattattctgagtccaagctaggcccttttgctaatcatgttcatacctcttatcttcctcccacagctcctgggcaacgtgctggtctgtgtgctggcccatcactttggcaaagaattgggataattactagatcgccaccatgagactgctggccttcctgagcctgctggccctggtgctgcaggagacaggcacctctgacacaggcagaccctttgtggaaatgtactctgagatccctgagatcatccacatgacagagggcagagagctggtcatcccctgcagagtgacaagccccaacatcacagtgaccctgaagaagttccctctggacacactgatccctgatggcaagagaatcatctgggacagcagaaagggcttcatcatcagcaatgccacctacaaagagattggcctgctgacctgtgaagccacagtgaatggccacctgtacaagaccaactacctgacacacagacagaccaacaccatcattgatgtggtgctgagccccagccatggcattgagctgtctgtgggagagaagctggtgctgaactgcacagccagaacagagctgaatgtgggcattgacttcaactgggagtaccccagcagcaagcaccagcacaagaaactggtcaacagggacctgaaaacccagagtggctctgagatgaagaaattcctgagcaccctgaccattgatggggtcaccagatctgaccagggcctgtacacatgtgctgccagctctggactgatgaccaagaaaaacagcacctttgtcagagtgcatgagaaggacaagacccacacctgtcctccatgtcctgcacctgagctgcttggaggcccctctgtgttcctgtttcctccaaagcctaaggacaccctgatgatcagcagaacacctgaagtgacctgtgtggtggtggatgtgtcccatgaggacccagaagtgaagttcaattggtatgtggatggggttgaagtgcacaatgccaagaccaagcctagagaggaacagtacaactccacctacagagtggtgtcagtgctgacagtgctgcaccaggactggctgaatggcaaagagtacaagtgcaaggtgtccaacaaggccctgcctgctcctattgagaaaaccatctccaaggccaagggccagcctagggaaccccaggtttacacactgccacctagcagggatgagctgacaaagaaccaggtgtccctgacctgcctggtcaagggcttctacccctctgacattgctgtggaatgggagagcaatggccagcctgagaacaactacaagacaacccctcctgtgctggactctgatggctcattcttcctgtacagcaagctgactgtggacaagagcagatggcagcagggaaatgtgttcagctgctctgtgatgcatgaggccctgcacaaccactacacccagaaaagcctgagcctgtctcctggcaagtgagcggccgcaagcttcgggtggcatccctgtgacccctccccagtgcctctcctggccctggaagttgccactccagtgcccaccagccttgtcctaataaaattaagttgcatcattttgtctgactaggtgtccttctataatattatggggtggaggggggtggtatggagcaaggggcaagttgggaagacaacctgtagggcctgcggggtctattgggaaccaagctggagtgcagtggcacaatcttggctcactgcaatctccgcctcctgggttcaagcgattctcctgcctcagcctcccgagttgttgggattccaggcatgcatgaccaggctcagctaatttttgtttttttggtagagacggggtttcaccatattggccaggctggtctccaactcctaatctcaggtgatctacccaccttggcctcccaaattgctgggattacaggcgtgaaccactgctcccttccctgtccttcgg

SEQ ID NO: 39 - DNA, 2743 bp, synthetic construct
  source 1..2743: mol_type = other DNA
acgcgtctagttattaatagtaatcaattacggggtcattagttcatagcccatatatggagttccgcgttacataacttacggtaaatggcccgcctggctgaccgcccaacgacccccgcccattgacgtcaataatgacgtatgttcccatagtaacgccaatagggactttccattgacgtcaatgggtggagtatttacggtaaactgcccacttggcagtacatcaagtgtatcatatgccaagtacgccccctattgacgtcaatgacggtaaatggcccgcctggcattatgcccagtacatgaccttacgggactttcctacttggcagtacatctacgtattagtcatcgctattaccatggtcgaggtgagccccacgttctgcttcactctccccatctcccccccctccccacccccaattttgtatttatttattttttaattattttgtgcagcgatgggggcggggggggggggggcgcgcgccaggcggggcggggcggggcgaggggcggggcggggcgaggcggagaggtgcggcggcagccaatcagagcggcgcgctccgaaagtttccttttatggcgaggcggcggcggcggcggccctataaaaagcgaagcgcgcggcgggcggggagtcgctgcgttgccttcgccccgtgccccgctccgcgccgcctcgcgccgcccgccccggctctgactgaccgcgttactcccacaggtgagcgggcgggacggcccttctcctccgggctgtaattagcaagaggtaagggtttaagggatggttggttggtggggtattaatgtttaattacctgttttacaggcctgaaatcacttggttttaggttggaattactagatcgccaccatgagactgctggccttcctgagcctgctggccctggtgctgcaggagacaggcacctctgacacaggcagaccctttgtggaaatgtactctgagatccctgagatcatccacatgacagagggcagagagctggtcatcccctgcagagtgacaagccccaacatcacagtgaccctgaagaagttccctctggacacactgatccctgatggcaagagaatcatctgggacagcagaaagggcttcatcatcagcaatgccacctacaaagagattggcctgctgacctgtgaagccacagtgaatggccacctgtacaagaccaactacctgacacacagacagaccaacaccatcattgatgtggtgctgagccccagccatggcattgagctgtctgtgggagagaagctggtgctgaactgcacagccagaacagagctgaatgtgggcattgacttcaactgggagtaccccagcagcaagcaccagcacaagaaactggtcaacagggacctgaaaacccagagtggctctgagatgaagaaattcctgagcaccctgaccattgatggggtcaccagatctgaccagggcctgtacacatgtgctgccagctctggactgatgaccaagaaaaacagcacctttgtcagagtgcatgagaaggacaagacccacacctgtcctccatgtcctgcacctgagctgcttggaggcccctctgtgttcctgtttcctccaaagcctaaggacaccctgatgatcagcagaacacctgaagtgacctgtgtggtggtggatgtgtcccatgaggacccagaagtgaagttcaattggtatgtggatggggttgaagtgcacaatgccaagaccaagcctagagaggaacagtacaactccacctacagagtggtgtcagtgctgacagtgctgcaccaggactggctgaatggcaaagagtacaagtgcaaggtgtccaacaaggccctgcctgctcctattgagaaaaccatctccaaggccaagggccagcctagggaaccccaggtttacacactgccacctagcagggatgagctgacaaagaaccaggtgtccctgacctgcctggtcaagggcttctacccctctgacattgctgtggaatgggagagcaatggccagcctgagaacaactacaagacaacccctcctgtgctggactctgatggctcattcttcctgtacagcaagctgactgtggacaagagcagatggcagcagggaaatgtgttcagctgctctgtgatgcatgaggccctgcacaaccactacacccagaaaagcctgagcctgtctcctggcaagtgagcggccgcaagcttcgggtggcatccctgtgacccctccccagtgcctctcctggccctggaagttgccactccagtgcccaccagccttgtcctaataaaattaagttgcatcattttgtctgactaggtgtccttctataatattatggggtggaggggggtggtatggagcaaggggcaagttgggaagacaacctgtagggcctgcggggtctattgggaaccaagctggagtgcagtggcacaatcttggctcactgcaatctccgcctcctgggttcaagcgattctcctgcctcagcctcccgagttgttgggattccaggcatgcatgaccaggctcagctaatttttgtttttttggtagagacggggtttcaccatattggccaggctggtctccaactcctaatctcaggtgatctacccaccttggcctcccaaattgctgggattacaggcgtgaaccactgctcccttccctgtccttcgg

SEQ ID NO: 40 - DNA, 3583 bp, synthetic construct
  source 1..3583: mol_type = other DNA
acgcgtctagttattaatagtaatcaattacggggtcattagttcatagcccatatatggagttccgcgttacataacttacggtaaatggcccgcctggctgaccgcccaacgacccccgcccattgacgtcaataatgacgtatgttcccatagtaacgccaatagggactttccattgacgtcaatgggtggagtatttacggtaaactgcccacttggcagtacatcaagtgtatcatatgccaagtacgccccctattgacgtcaatgacggtaaatggcccgcctggcattatgcccagtacatgaccttacgggactttcctacttggcagtacatctacgtattagtcatcgctattaccatggtcgaggtgagccccacgttctgcttcactctccccatctcccccccctccccacccccaattttgtatttatttattttttaattattttgtgcagcgatgggggcggggggggggggggcgcgcgccaggcggggcggggcggggcgaggggcggggcggggcgaggcggagaggtgcggcggcagccaatcagagcggcgcgctccgaaagtttccttttatggcgaggcggcggcggcggcggccctataaaaagcgaagcgcgcggcgggcgggagtcgctgcgcgctgccttcgccccgtgccccgctccgccgccgcctcgcgccgcccgccccggctctgactgaccgcgttactcccacaggtgagcgggcgggacggcccttctcctccgggctgtaattagcgcttggtttaatgacggcttgtttcttttctgtggctgcgtgaaagccttgaggggctccgggagggccctttgtgcggggggagcggctcggggggtgcgtgcgtgtgtgtgtgcgtggggagcgccgcgtgcggctccgcgctgcccggcggctgtgagcgctgcgggcgcggcgcggggctttgtgcgctccgcagtgtgcgcgaggggagcgcggccgggggcggtgccccgcggtgcggggggggctgcgaggggaacaaaggctgcgtgcggggtgtgtgcgtgggggggtgagcagggggtgtgggcgcgtcggtcgggctgcaaccccccctgcacccccctccccgagttgctgagcacggcccggcttcgggtgcggggctccgtacggggcgtggcgcggggctcgccgtgccgggcggggggtggcggcaggtgggggtgccgggcggggcggggccgcctcgggccggggagggctcgggggaggggcgcggcggcccccggagcgccggcggctgtcgaggcgcggcgagccgcagccattgccttttatggtaatcgtgcgagagggcgcagggacttcctttgtcccaaatctgtgcggagccgaaatctgggaggcgccgccgcaccccctctagcgggcgcggggcgaagcggtgcggcgccggcaggaaggaaatgggcggggagggccttcgtgcgtcgccgcgccgccgtccccttctccctctccagcctcggggctgtccgcggggggacggctgccttcgggggggacggggcagggcggggttcggcttctggcgtgtgaccggcggctctagagcctctgctaaccatgttcatgccttcttctttttcctacagctcctgggcaacgtgctggttattgtgctgtctcatcattttggcaaagaattactagatcgccaccatgagactgctggccttcctgagcctgctggccctggtgctgcaggagacaggcacctctgacacaggcagaccctttgtggaaatgtactctgagatccctgagatcatccacatgacagagggcagagagctggtcatcccctgcagagtgacaagccccaacatcacagtgaccctgaagaagttccctctggacacactgatccctgatggcaagagaatcatctgggacagcagaaagggcttcatcatcagcaatgccacctacaaagagattggcctgctgacctgtgaagccacagtgaatggccacctgtacaagaccaactacctgacacacagacagaccaacaccatcattgatgtggtgctgagccccagccatggcattgagctgtctgtgggagagaagctggtgctgaactgcacagccagaacagagctgaatgtgggcattgacttcaactgggagtaccccagcagcaagcaccagcacaagaaactggtcaacagggacctgaaaacccagagtggctctgagatgaagaaattcctgagcaccctgaccattgatggggtcaccagatctgaccagggcctgtacacatgtgctgccagctctggactgatgaccaagaaaaacagcacctttgtcagagtgcatgagaaggacaagacccacacctgtcctccatgtcctgcacctgagctgcttggaggcccctctgtgttcctgtttcctccaaagcctaaggacaccctgatgatcagcagaacacctgaagtgacctgtgtggtggtggatgtgtcccatgaggacccagaagtgaagttcaattggtatgtggatggggttgaagtgcacaatgccaagaccaagcctagagaggaacagtacaactccacctacagagtggtgtcagtgctgacagtgctgcaccaggactggctgaatggcaaagagtacaagtgcaaggtgtccaacaaggccctgcctgctcctattgagaaaaccatctccaaggccaagggccagcctagggaaccccaggtttacacactgccacctagcagggatgagctgacaaagaaccaggtgtccctgacctgcctggtcaagggcttctacccctctgacattgctgtggaatgggagagcaatggccagcctgagaacaactacaagacaacccctcctgtgctggactctgatggctcattcttcctgtacagcaagctgactgtggacaagagcagatggcagcagggaaatgtgttcagctgctctgtgatgcatgaggccctgcacaaccactacacccagaaaagcctgagcctgtctcctggcaagtgagcggccgcaagcttcgggtggcatccctgtgacccctccccagtgcctctcctggccctggaagttgccactccagtgcccaccagccttgtcctaataaaattaagttgcatcattttgtctgactaggtgtccttctataatattatggggtggaggggggtggtatggagcaaggggcaagttgggaagacaacctgtagggcctgcggggtctattgggaaccaagctggagtgcagtggcacaatcttggctcactgcaatctccgcctcctgggttcaagcgattctcctgcctcagcctcccgagttgttgggattccaggcatgcatgaccaggctcagctaatttttgtttttttggtagagacggggtttcaccatattggccaggctggtctccaactcctaatctcaggtgatctacccaccttggcctcccaaattgctgggattacaggcgtgaaccactgctcccttccctgtccttcgg

SEQ ID NO: 41 - DNA, 3059 bp, synthetic construct
  source 1..3059: mol_type = other DNA
acgcgtctagttattaatagtaatcaattacggggtcattagttcatagcccatatatggagttccgcgttacataacttacggtaaatggcccgcctggctgaccgcccaacgacccccgcccattgacgtcaataatgacgtatgttcccatagtaacgccaatagggactttccattgacgtcaatgggtggagtatttacggtaaactgcccacttggcagtacatcaagtgtatcatatgccaagtacgccccctattgacgtcaatgacggtaaatggcccgcctggcattatgcccagtacatgaccttatgggactttcctacttggcagtacatctacgtattagtcatcgctattaccatggtgatgcggttttggcagtacatcaatgggcgtggatagcggtttgactcacggggatttccaagtctccaccccattgacgtcaatgggagtttgttttggcaccaaaatcaacgggactttccaaaatgtcgtaacaactccgccccattgacgcaaatgggcggtaggcgtgtacggtgggaggtctatataagcagagctcgtttagtgaaccgtcagatcgcctggagacgccatccacgctgttttgacctccatagaagacaccgggaccgatccagcctccgcggattcgaatcccggccgggaacggtgcattggaacgcggattccccgtgccaagagtgacgtaagtaccgcctatagagtctataggcccacaaaaaatgctttcttcttttaatatacttttttgtttatcttatttctaatactttccctaatctctttctttcagggcaataatgatacaatgtatcatgcctctttgcaccattctaaagaataacagtgataatttctgggttaaggcaatagcaatatttctgcatataaatatttctgcatataaattgtaactgatgtaagaggtttcatattgctaatagcagctacaatccagctaccattctgcttttattttatggttgggataaggctggattattctgagtccaagctaggcccttttgctaatcatgttcatacctcttatcttcctcccacagctcctgggcaacgtgctggtctgtgtgctggcccatcactttggcaaagaattgggataattactagatcgccaccatgcacagacccagaaggaggggcaccagacctccacctctggctctgctggcagccctgctgctggcagctagaggagcagatgcctctgacacaggcagaccctttgtggaaatgtactctgagatccctgagatcatccacatgacagagggcagagagctggtcatcccctgcagagtgacaagccccaacatcacagtgaccctgaagaagttccctctggacacactgatccctgatggcaagagaatcatctgggacagcagaaagggcttcatcatcagcaatgccacctacaaagagattggcctgctgacctgtgaagccacagtgaatggccacctgtacaagaccaactacctgacacacagacagaccaacaccatcattgatgtggtgctgagccccagccatggcattgagctgtctgtgggagagaagctggtgctgaactgcacagccagaacagagctgaatgtgggcattgacttcaactgggagtaccccagcagcaagcaccagcacaagaaactggtcaacagggacctgaaaacccagagtggctctgagatgaagaaattcctgagcaccctgaccattgatggggtcaccagatctgaccagggcctgtacacatgtgctgccagctctggactgatgaccaagaaaaacagcacctttgtcagagtgcatgagaaggacaagacccacacctgtcctccatgtcctgcacctgagctgcttggaggcccctctgtgttcctgtttcctccaaagcctaaggacaccctgatgatcagcagaacacctgaagtgacctgtgtggtggtggatgtgtcccatgaggacccagaagtgaagttcaattggtatgtggatggggttgaagtgcacaatgccaagaccaagcctagagaggaacagtacaactccacctacagagtggtgtcagtgctgacagtgctgcaccaggactggctgaatggcaaagagtacaagtgcaaggtgtccaacaaggccctgcctgctcctattgagaaaaccatctccaaggccaagggccagcctagggaaccccaggtttacacactgccacctagcagggatgagctgacaaagaaccaggtgtccctgacctgcctggtcaagggcttctacccctctgacattgctgtggaatgggagagcaatggccagcctgagaacaactacaagacaacccctcctgtgctggactctgatggctcattcttcctgtacagcaagctgactgtggacaagagcagatggcagcagggaaatgtgttcagctgctctgtgatgcatgaggccctgcacaaccactacacccagaaaagcctgagcctgtctcctggcaagtgagcggccgcaagcttcgggtggcatccctgtgacccctccccagtgcctctcctggccctggaagttgccactccagtgcccaccagccttgtcctaataaaattaagttgcatcattttgtctgactaggtgtccttctataatattatggggtggaggggggtggtatggagcaaggggcaagttgggaagacaacctgtagggcctgcggggtctattgggaaccaagctggagtgcagtggcacaatcttggctcactgcaatctccgcctcctgggttcaagcgattctcctgcctcagcctcccgagttgttgggattccaggcatgcatgaccaggctcagctaatttttgtttttttggtagagacggggtttcaccatattggccaggctggtctccaactcctaatctcaggtgatctacccaccttggcctcccaaattgctgggattacaggcgtgaaccactgctcccttccctgtccttcgg

SEQ ID NO: 42 - DNA, 2773 bp, synthetic construct
  source 1..2773: mol_type = other DNA
acgcgtctagttattaatagtaatcaattacggggtcattagttcatagcccatatatggagttccgcgttacataacttacggtaaatggcccgcctggctgaccgcccaacgacccccgcccattgacgtcaataatgacgtatgttcccatagtaacgccaatagggactttccattgacgtcaatgggtggagtatttacggtaaactgcccacttggcagtacatcaagtgtatcatatgccaagtacgccccctattgacgtcaatgacggtaaatggcccgcctggcattatgcccagtacatgaccttacgggactttcctacttggcagtacatctacgtattagtcatcgctattaccatggtcgaggtgagccccacgttctgcttcactctccccatctcccccccctccccacccccaattttgtatttatttattttttaattattttgtgcagcgatgggggcggggggggggggggcgcgcgccaggcggggcggggcggggcgaggggcggggcggggcgaggcggagaggtgcggcggcagccaatcagagcggcgcgctccgaaagtttccttttatggcgaggcggcggcggcggcggccctataaaaagcgaagcgcgcggcgggcggggagtcgctgcgttgccttcgccccgtgccccgctccgcgccgcctcgcgccgcccgccccggctctgactgaccgcgttactcccacaggtgagcgggcgggacggcccttctcctccgggctgtaattagcaagaggtaagggtttaagggatggttggttggtggggtattaatgtttaattacctgttttacaggcctgaaatcacttggttttaggttggaattactagatcgccaccatgcacagacccagaaggaggggcaccagacctccacctctggctctgctggcagccctgctgctggcagctagaggagcagatgcctctgacacaggcagaccctttgtggaaatgtactctgagatccctgagatcatccacatgacagagggcagagagctggtcatcccctgcagagtgacaagccccaacatcacagtgaccctgaagaagttccctctggacacactgatccctgatggcaagagaatcatctgggacagcagaaagggcttcatcatcagcaatgccacctacaaagagattggcctgctgacctgtgaagccacagtgaatggccacctgtacaagaccaactacctgacacacagacagaccaacaccatcattgatgtggtgctgagccccagccatggcattgagctgtctgtgggagagaagctggtgctgaactgcacagccagaacagagctgaatgtgggcattgacttcaactgggagtaccccagcagcaagcaccagcacaagaaactggtcaacagggacctgaaaacccagagtggctctgagatgaagaaattcctgagcaccctgaccattgatggggtcaccagatctgaccagggcctgtacacatgtgctgccagctctggactgatgaccaagaaaaacagcacctttgtcagagtgcatgagaaggacaagacccacacctgtcctccatgtcctgcacctgagctgcttggaggcccctctgtgttcctgtttcctccaaagcctaaggacaccctgatgatcagcagaacacctgaagtgacctgtgtggtggtggatgtgtcccatgaggacccagaagtgaagttcaattggtatgtggatggggttgaagtgcacaatgccaagaccaagcctagagaggaacagtacaactccacctacagagtggtgtcagtgctgacagtgctgcaccaggactggctgaatggcaaagagtacaagtgcaaggtgtccaacaaggccctgcctgctcctattgagaaaaccatctccaaggccaagggccagcctagggaaccccaggtttacacactgccacctagcagggatgagctgacaaagaaccaggtgtccctgacctgcctggtcaagggcttctacccctctgacattgctgtggaatgggagagcaatggccagcctgagaacaactacaagacaacccctcctgtgctggactctgatggctcattcttcctgtacagcaagctgactgtggacaagagcagatggcagcagggaaatgtgttcagctgctctgtgatgcatgaggccctgcacaaccactacacccagaaaagcctgagcctgtctcctggcaagtgagcggccgcaagcttcgggtggcatccctgtgacccctccccagtgcctctcctggccctggaagttgccactccagtgcccaccagccttgtcctaataaaattaagttgcatcattttgtctgactaggtgtccttctataatattatggggtggaggggggtggtatggagcaaggggcaagttgggaagacaacctgtagggcctgcggggtctattgggaaccaagctggagtgcagtggcacaatcttggctcactgcaatctccgcctcctgggttcaagcgattctcctgcctcagcctcccgagttgttgggattccaggcatgcatgaccaggctcagctaatttttgtttttttggtagagacggggtttcaccatattggccaggctggtctccaactcctaatctcaggtgatctacccaccttggcctcccaaattgctgggattacaggcgtgaaccactgctcccttccctgtccttcgg

SEQ ID NO: 43 - DNA, 3613 bp, synthetic construct
  source 1..3613: mol_type = other DNA
acgcgtctagttattaatagtaatcaattacggggtcattagttcatagcccatatatggagttccgcgttacataacttacggtaaatggcccgcctggctgaccgcccaacgacccccgcccattgacgtcaataatgacgtatgttcccatagtaacgccaatagggactttccattgacgtcaatgggtggagtatttacggtaaactgcccacttggcagtacatcaagtgtatcatatgccaagtacgccccctattgacgtcaatgacggtaaatggcccgcctggcattatgcccagtacatgaccttacgggactttcctacttggcagtacatctacgtattagtcatcgctattaccatggtcgaggtgagccccacgttctgcttcactctccccatctcccccccctccccacccccaattttgtatttatttattttttaattattttgtgcagcgatgggggcggggggggggggggcgcgcgccaggcggggcggggcggggcgaggggcggggcggggcgaggcggagaggtgcggcggcagccaatcagagcggcgcgctccgaaagtttccttttatggcgaggcggcggcggcggcggccctataaaaagcgaagcgcgcggcgggcgggagtcgctgcgcgctgccttcgccccgtgccccgctccgccgccgcctcgcgccgcccgccccggctctgactgaccgcgttactcccacaggtgagcgggcgggacggcccttctcctccgggctgtaattagcgcttggtttaatgacggcttgtttcttttctgtggctgcgtgaaagccttgaggggctccgggagggccctttgtgcggggggagcggctcggggggtgcgtgcgtgtgtgtgtgcgtggggagcgccgcgtgcggctccgcgctgcccggcggctgtgagcgctgcgggcgcggcgcggggctttgtgcgctccgcagtgtgcgcgaggggagcgcggccgggggcggtgccccgcggtgcggggggggctgcgaggggaacaaaggctgcgtgcggggtgtgtgcgtgggggggtgagcagggggtgtgggcgcgtcggtcgggctgcaaccccccctgcacccccctccccgagttgctgagcacggcccggcttcgggtgcggggctccgtacggggcgtggcgcggggctcgccgtgccgggcggggggtggcggcaggtgggggtgccgggcggggcggggccgcctcgggccggggagggctcgggggaggggcgcggcggcccccggagcgccggcggctgtcgaggcgcggcgagccgcagccattgccttttatggtaatcgtgcgagagggcgcagggacttcctttgtcccaaatctgtgcggagccgaaatctgggaggcgccgccgcaccccctctagcgggcgcggggcgaagcggtgcggcgccggcaggaaggaaatgggcggggagggccttcgtgcgtcgccgcgccgccgtccccttctccctctccagcctcggggctgtccgcggggggacggctgccttcgggggggacggggcagggcggggttcggcttctggcgtgtgaccggcggctctagagcctctgctaaccatgttcatgccttcttctttttcctacagctcctgggcaacgtgctggttattgtgctgtctcatcattttggcaaagaattactagatcgccaccatgcacagacccagaaggaggggcaccagacctccacctctggctctgctggcagccctgctgctggcagctagaggagcagatgcctctgacacaggcagaccctttgtggaaatgtactctgagatccctgagatcatccacatgacagagggcagagagctggtcatcccctgcagagtgacaagccccaacatcacagtgaccctgaagaagttccctctggacacactgatccctgatggcaagagaatcatctgggacagcagaaagggcttcatcatcagcaatgccacctacaaagagattggcctgctgacctgtgaagccacagtgaatggccacctgtacaagaccaactacctgacacacagacagaccaacaccatcattgatgtggtgctgagccccagccatggcattgagctgtctgtgggagagaagctggtgctgaactgcacagccagaacagagctgaatgtgggcattgacttcaactgggagtaccccagcagcaagcaccagcacaagaaactggtcaacagggacctgaaaacccagagtggctctgagatgaagaaattcctgagcaccctgaccattgatggggtcaccagatctgaccagggcctgtacacatgtgctgccagctctggactgatgaccaagaaaaacagcacctttgtcagagtgcatgagaaggacaagacccacacctgtcctccatgtcctgcacctgagctgcttggaggcccctctgtgttcctgtttcctccaaagcctaaggacaccctgatgatcagcagaacacctgaagtgacctgtgtggtggtggatgtgtcccatgaggacccagaagtgaagttcaattggtatgtggatggggttgaagtgcacaatgccaagaccaagcctagagaggaacagtacaactccacctacagagtggtgtcagtgctgacagtgctgcaccaggactggctgaatggcaaagagtacaagtgcaaggtgtccaacaaggccctgcctgctcctattgagaaaaccatctccaaggccaagggccagcctagggaaccccaggtttacacactgccacctagcagggatgagctgacaaagaaccaggtgtccctgacctgcctggtcaagggcttctacccctctgacattgctgtggaatgggagagcaatggccagcctgagaacaactacaagacaacccctcctgtgctggactctgatggctcattcttcctgtacagcaagctgactgtggacaagagcagatggcagcagggaaatgtgttcagctgctctgtgatgcatgaggccctgcacaaccactacacccagaaaagcctgagcctgtctcctggcaagtgagcggccgcaagcttcgggtggcatccctgtgacccctccccagtgcctctcctggccctggaagttgccactccagtgcccaccagccttgtcctaataaaattaagttgcatcattttgtctgactaggtgtccttctataatattatggggtggaggggggtggtatggagcaaggggcaagttgggaagacaacctgtagggcctgcggggtctattgggaaccaagctggagtgcagtggcacaatcttggctcactgcaatctccgcctcctgggttcaagcgattctcctgcctcagcctcccgagttgttgggattccaggcatgcatgaccaggctcagctaatttttgtttttttggtagagacggggtttcaccatattggccaggctggtctccaactcctaatctcaggtgatctacccaccttggcctcccaaattgctgggattacaggcgtgaaccactgctcccttccctgtccttcgg

SEQ ID NO: 44 - protein, 18 aa, synthetic construct
MKWVTFISLLFLFSSAYS

SEQ ID NO: 45 - protein, 19 aa, synthetic construct
MRLLAFLSLLALVLQETGT

SEQ ID NO: 46 - protein, 20 aa, synthetic construct
MYRMQLLSCIALSLALVTNS

SEQ ID NO: 47 - protein, 29 aa, synthetic construct
MHRPRRRGTRPPPLALLAALLLAARGADA

SEQ ID NO: 48 - protein, 432 aa, synthetic construct
SDTGRPFVEMYSEIPEIIHMTEGRELVIPCRVTSPNITVTLKKFPLDTLIPDGKRIIWDSRKGFIISNATYKEIGLLTCEATVNGHLYKTNYLTHRQTNTIIDVVLSPSHGIELSVGEKLVLNCTARTELNVGIDFNWEYPSSKHQHKKLVNRDLKTQSGSEMKKFLSTLTIDGVTRSDQGLYTCAASSGLMTKKNSTFVRVHEKDKTHTCPPCPAPELLGGPSVFLFPPKPKDTLMISRTPEVTCVVVDVSHEDPEVKFNWYVDGVEVHNAKTKPREEQYNSTYRVVSVLTVLHQDWLNGKEYKCKVSNKALPAPIEKTISKAKGQPREPQVYTLPPSRDELTKNQVSLTCLVKGFYPSDIAVEWESNGQPENNYKTTPPVLDSDGSFFLYSKLTVDKSRWQQGNVFSCSVMHEALHNHYTQKSLSLSPGK

SEQ ID NO: 49 - DNA, 3618 bp, synthetic construct
  source 1..3618: mol_type = other DNA
ttggccactccctctctgcgcgctcgctcgctcactgaggccgggcgaccaaaggtcgcccgacgcccgggctttgcccgggcggcctcagtgagcgagcgagcgcgcagagagggagtggccaactccatcactaggggttcctctcgagacgcgtctagttattaatagtaatcaattacggggtcattagttcatagcccatatatggagttccgcgttacataacttacggtaaatggcccgcctggctgaccgcccaacgacccccgcccattgacgtcaataatgacgtatgttcccatagtaacgccaatagggactttccattgacgtcaatgggtggagtatttacggtaaactgcccacttggcagtacatcaagtgtatcatatgccaagtacgccccctattgacgtcaatgacggtaaatggcccgcctggcattatgcccagtacatgaccttatgggactttcctacttggcagtacatctacgtattagtcatcgctattaccatggtgatgcggttttggcagtacatcaatgggcgtggatagcggtttgactcacggggatttccaagtctccaccccattgacgtcaatgggagtttgttttggcaccaaaatcaacgggactttccaaaatgtcgtaacaactccgccccattgacgcaaatgggcggtaggcgtgtacggtgggaggtctatataagcagagctcgtttagtgaaccgtcagatcgcctggagacgccatccacgctgttttgacctccatagaagacaccgggaccgatccagcctccgcggattcgaatcccggccgggaacggtgcattggaacgcggattccccgtgccaagagtgacgtaagtaccgcctatagagtctataggcccacaaaaaatgctttcttcttttaatatacttttttgtttatcttatttctaatactttccctaatctctttctttcagggcaataatgatacaatgtatcatgcctctttgcaccattctaaagaataacagtgataatttctgggttaaggcaatagcaatatttctgcatataaatatttctgcatataaattgtaactgatgtaagaggtttcatattgctaatagcagctacaatccagctaccattctgcttttattttatggttgggataaggctggattattctgagtccaagctaggcccttttgctaatcatgttcatacctcttatcttcctcccacagctcctgggcaacgtgctggtctgtgtgctggcccatcactttggcaaagaattgggataattactagatcatggaagatgccaaaaacattaagaagggcccagcgccattctacccactcgaagacgggaccgccggcgagcagctgcacaaagccatgaagcgctacgccctggtgcccggcaccatcgcctttaccgacgcacatatcgaggtggacattacctacgccgagtacttcgagatgagcgttcggctggcagaagctatgaagcgctatgggctgaatacaaaccatcggatcgtggtgtgcagcgagaatagcttgcagttcttcatgcccgtgttgggtgccctgttcatcggtgtggctgtggccccagctaacgacatctacaacgagcgcgagctgctgaacagcatgggcatcagccagcccaccgtcgtattcgtgagcaagaaagggctgcaaaagatcctcaacgtgcaaaagaagctaccgatcatacaaaagatcatcatcatggatagcaagaccgactaccagggcttccaaagcatgtacaccttcgtgacttcccatttgccacccggcttcaacgagtacgacttcgtgcccgagagcttcgaccgggacaaaaccatcgccctgatcatgaacagtagtggcagtaccggattgcccaagggcgtagccctaccgcaccgcaccgcttgtgtccgattcagtcatgcccgcgaccccatcttcggcaaccagatcatccccgacaccgctatcctcagcgtggtgccatttcaccacggcttcggcatgttcaccacgctgggctacttgatctgcggctttcgggtcgtgctcatgtaccgcttcgaggaggagctattcttgcgcagcttgcaagactataagattcaatctgccctgctggtgcccacactatttagcttcttcgctaagagcactctcatcgacaagtacgacctaagcaacttgcacgagatcgccagcggcggggcgccgctcagcaaggaggtaggtgaggccgtggccaaacgcttccacctaccaggcatccgccagggctacggcctgacagaaacaaccagcgccattctgatcacccccgaaggggacgacaagcctggcgcagtaggcaaggtggtgcccttcttcgaggctaaggtggtggacttggacaccggtaagacactgggtgtgaaccagcgcggcgagctgtgcgtccgtggccccatgatcatgagcggctacgttaacaaccccgaggctacaaacgctctcatcgacaaggacggctggctgcacagcggcgacatcgcctactgggacgaggacgagcacttcttcatcgtggaccggctgaagagcctgatcaaatacaagggctaccaggtagccccagccgaactggagagcatcctgctgcaacaccccaacatcttcgacgccggggtcgccggcctgcccgacgacgatgccggcgagctgcccgccgcagtcgtcgtgctggaacacggtaaaaccatgaccgagaaggagatcgtggactatgtggccagccaggttacaaccgccaagaagctgcgcggtggtgttgtgttcgtggacgaggtgcctaaaggactgaccggcaagttggacgcccgcaagatccgcgagattctcattaaggccaagaagggcggcaagatcgccgtgtaagcggccgcaagcttcgggtggcatccctgtgacccctccccagtgcctctcctggccctggaagttgccactccagtgcccaccagccttgtcctaataaaattaagttgcatcattttgtctgactaggtgtccttctataatattatggggtggaggggggtggtatggagcaaggggcaagttgggaagacaacctgtagggcctgcggggtctattgggaaccaagctggagtgcagtggcacaatcttggctcactgcaatctccgcctcctgggttcaagcgattctcctgcctcagcctcccgagttgttgggattccaggcatgcatgaccaggctcagctaatttttgtttttttggtagagacggggtttcaccatattggccaggctggtctccaactcctaatctcaggtgatctacccaccttggcctcccaaattgctgggattacaggcgtgaaccactgctcccttccctgtccttcggtctagaaggaacccctagtgatggagttggccactccctctctgcgcgctcgctcgctcactgaggccgggcgaccaaaggtcgcccgacgcccgggctttgcccgggcggcctcagtgagcgagcgagcgcgcagagagggagtgg

SEQ ID NO: 50 - DNA, 3332 bp, synthetic construct
  source 1..3332: mol_type = other DNA
ttggccactccctctctgcgcgctcgctcgctcactgaggccgggcgaccaaaggtcgcccgacgcccgggctttgcccgggcggcctcagtgagcgagcgagcgcgcagagagggagtggccaactccatcactaggggttcctctcgagacgcgtctagttattaatagtaatcaattacggggtcattagttcatagcccatatatggagttccgcgttacataacttacggtaaatggcccgcctggctgaccgcccaacgacccccgcccattgacgtcaataatgacgtatgttcccatagtaacgccaatagggactttccattgacgtcaatgggtggagtatttacggtaaactgcccacttggcagtacatcaagtgtatcatatgccaagtacgccccctattgacgtcaatgacggtaaatggcccgcctggcattatgcccagtacatgaccttacgggactttcctacttggcagtacatctacgtattagtcatcgctattaccatggtcgaggtgagccccacgttctgcttcactctccccatctcccccccctccccacccccaattttgtatttatttattttttaattattttgtgcagcgatgggggcggggggggggggggcgcgcgccaggcggggcggggcggggcgaggggcggggcggggcgaggcggagaggtgcggcggcagccaatcagagcggcgcgctccgaaagtttccttttatggcgaggcggcggcggcggcggccctataaaaagcgaagcgcgcggcgggcggggagtcgctgcgttgccttcgccccgtgccccgctccgcgccgcctcgcgccgcccgccccggctctgactgaccgcgttactcccacaggtgagcgggcgggacggcccttctcctccgggctgtaattagcaagaggtaagggtttaagggatggttggttggtggggtattaatgtttaattacctgttttacaggcctgaaatcacttggttttaggttggaattactagatcatggaagatgccaaaaacattaagaagggcccagcgccattctacccactcgaagacgggaccgccggcgagcagctgcacaaagccatgaagcgctacgccctggtgcccggcaccatcgcctttaccgacgcacatatcgaggtggacattacctacgccgagtacttcgagatgagcgttcggctggcagaagctatgaagcgctatgggctgaatacaaaccatcggatcgtggtgtgcagcgagaatagcttgcagttcttcatgcccgtgttgggtgccctgttcatcggtgtggctgtggccccagctaacgacatctacaacgagcgcgagctgctgaacagcatgggcatcagccagcccaccgtcgtattcgtgagcaagaaagggctgcaaaagatcctcaacgtgcaaaagaagctaccgatcatacaaaagatcatcatcatggatagcaagaccgactaccagggcttccaaagcatgtacaccttcgtgacttcccatttgccacccggcttcaacgagtacgacttcgtgcccgagagcttcgaccgggacaaaaccatcgccctgatcatgaacagtagtggcagtaccggattgcccaagggcgtagccctaccgcaccgcaccgcttgtgtccgattcagtcatgcccgcgaccccatcttcggcaaccagatcatccccgacaccgctatcctcagcgtggtgccatttcaccacggcttcggcatgttcaccacgctgggctacttgatctgcggctttcgggtcgtgctcatgtaccgcttcgaggaggagctattcttgcgcagcttgcaagactataagattcaatctgccctgctggtgcccacactatttagcttcttcgctaagagcactctcatcgacaagtacgacctaagcaacttgcacgagatcgccagcggcggggcgccgctcagcaaggaggtaggtgaggccgtggccaaacgcttccacctaccaggcatccgccagggctacggcctgacagaaacaaccagcgccattctgatcacccccgaaggggacgacaagcctggcgcagtaggcaaggtggtgcccttcttcgaggctaaggtggtggacttggacaccggtaagacactgggtgtgaaccagcgcggcgagctgtgcgtccgtggccccatgatcatgagcggctacgttaacaaccccgaggctacaaacgctctcatcgacaaggacggctggctgcacagcggcgacatcgcctactgggacgaggacgagcacttcttcatcgtggaccggctgaagagcctgatcaaatacaagggctaccaggtagccccagccgaactggagagcatcctgctgcaacaccccaacatcttcgacgccggggtcgccggcctgcccgacgacgatgccggcgagctgcccgccgcagtcgtcgtgctggaacacggtaaaaccatgaccgagaaggagatcgtggactatgtggccagccaggttacaaccgccaagaagctgcgcggtggtgttgtgttcgtggacgaggtgcctaaaggactgaccggcaagttggacgcccgcaagatccgcgagattctcattaaggccaagaagggcggcaagatcgccgtgtaagcggccgcaagcttcgggtggcatccctgtgacccctccccagtgcctctcctggccctggaagttgccactccagtgcccaccagccttgtcctaataaaattaagttgcatcattttgtctgactaggtgtccttctataatattatggggtggaggggggtggtatggagcaaggggcaagttgggaagacaacctgtagggcctgcggggtctattgggaaccaagctggagtgcagtggcacaatcttggctcactgcaatctccgcctcctgggttcaagcgattctcctgcctcagcctcccgagttgttgggattccaggcatgcatgaccaggctcagctaatttttgtttttttggtagagacggggtttcaccatattggccaggctggtctccaactcctaatctcaggtgatctacccaccttggcctcccaaattgctgggattacaggcgtgaaccactgctcccttccctgtccttcggtctagaaggaacccctagtgatggagttggccactccctctctgcgcgctcgctcgctcactgaggccgggcgaccaaaggtcgcccgacgcccgggctttgcccgggcggcctcagtgagcgagcgagcgcgcagagagggagtgg

SEQ ID NO: 51 - DNA, 4172 bp, synthetic construct
  source 1..4172: mol_type = other DNA
ttggccactccctctctgcgcgctcgctcgctcactgaggccgggcgaccaaaggtcgcccgacgcccgggctttgcccgggcggcctcagtgagcgagcgagcgcgcagagagggagtggccaactccatcactaggggttcctctcgagacgcgtctagttattaatagtaatcaattacggggtcattagttcatagcccatatatggagttccgcgttacataacttacggtaaatggcccgcctggctgaccgcccaacgacccccgcccattgacgtcaataatgacgtatgttcccatagtaacgccaatagggactttccattgacgtcaatgggtggagtatttacggtaaactgcccacttggcagtacatcaagtgtatcatatgccaagtacgccccctattgacgtcaatgacggtaaatggcccgcctggcattatgcccagtacatgaccttacgggactttcctacttggcagtacatctacgtattagtcatcgctattaccatggtcgaggtgagccccacgttctgcttcactctccccatctcccccccctccccacccccaattttgtatttatttattttttaattattttgtgcagcgatgggggcggggggggggggggcgcgcgccaggcggggcggggcggggcgaggggcggggcggggcgaggcggagaggtgcggcggcagccaatcagagcggcgcgctccgaaagtttccttttatggcgaggcggcggcggcggcggccctataaaaagcgaagcgcgcggcgggcgggagtcgctgcgcgctgccttcgccccgtgccccgctccgccgccgcctcgcgccgcccgccccggctctgactgaccgcgttactcccacaggtgagcgggcgggacggcccttctcctccgggctgtaattagcgcttggtttaatgacggcttgtttcttttctgtggctgcgtgaaagccttgaggggctccgggagggccctttgtgcggggggagcggctcggggggtgcgtgcgtgtgtgtgtgcgtggggagcgccgcgtgcggctccgcgctgcccggcggctgtgagcgctgcgggcgcggcgcggggctttgtgcgctccgcagtgtgcgcgaggggagcgcggccgggggcggtgccccgcggtgcggggggggctgcgaggggaacaaaggctgcgtgcggggtgtgtgcgtgggggggtgagcagggggtgtgggcgcgtcggtcgggctgcaaccccccctgcacccccctccccgagttgctgagcacggcccggcttcgggtgcggggctccgtacggggcgtggcgcggggctcgccgtgccgggcggggggtggcggcaggtgggggtgccgggcggggcggggccgcctcgggccggggagggctcgggggaggggcgcggcggcccccggagcgccggcggctgtcgaggcgcggcgagccgcagccattgccttttatggtaatcgtgcgagagggcgcagggacttcctttgtcccaaatctgtgcggagccgaaatctgggaggcgccgccgcaccccctctagcgggcgcggggcgaagcggtgcggcgccggcaggaaggaaatgggcggggagggccttcgtgcgtcgccgcgccgccgtccccttctccctctccagcctcggggctgtccgcggggggacggctgccttcgggggggacggggcagggcggggttcggcttctggcgtgtgaccggcggctctagagcctctgctaaccatgttcatgccttcttctttttcctacagctcctgggcaacgtgctggttattgtgctgtctcatcattttggcaaagaattactagatcatggaagatgccaaaaacattaagaagggcccagcgccattctacccactcgaagacgggaccgccggcgagcagctgcacaaagccatgaagcgctacgccctggtgcccggcaccatcgcctttaccgacgcacatatcgaggtggacattacctacgccgagtacttcgagatgagcgttcggctggcagaagctatgaagcgctatgggctgaatacaaaccatcggatcgtggtgtgcagcgagaatagcttgcagttcttcatgcccgtgttgggtgccctgttcatcggtgtggctgtggccccagctaacgacatctacaacgagcgcgagctgctgaacagcatgggcatcagccagcccaccgtcgtattcgtgagcaagaaagggctgcaaaagatcctcaacgtgcaaaagaagctaccgatcatacaaaagatcatcatcatggatagcaagaccgactaccagggcttccaaagcatgtacaccttcgtgacttcccatttgccacccggcttcaacgagtacgacttcgtgcccgagagcttcgaccgggacaaaaccatcgccctgatcatgaacagtagtggcagtaccggattgcccaagggcgtagccctaccgcaccgcaccgcttgtgtccgattcagtcatgcccgcgaccccatcttcggcaaccagatcatccccgacaccgctatcctcagcgtggtgccatttcaccacggcttcggcatgttcaccacgctgggctacttgatctgcggctttcgggtcgtgctcatgtaccgcttcgaggaggagctattcttgcgcagcttgcaagactataagattcaatctgccctgctggtgcccacactatttagcttcttcgctaagagcactctcatcgacaagtacgacctaagcaacttgcacgagatcgccagcggcggggcgccgctcagcaaggaggtaggtgaggccgtggccaaacgcttccacctaccaggcatccgccagggctacggcctgacagaaacaaccagcgccattctgatcacccccgaaggggacgacaagcctggcgcagtaggcaaggtggtgcccttcttcgaggctaaggtggtggacttggacaccggtaagacactgggtgtgaaccagcgcggcgagctgtgcgtccgtggccccatgatcatgagcggctacgttaacaaccccgaggctacaaacgctctcatcgacaaggacggctggctgcacagcggcgacatcgcctactgggacgaggacgagcacttcttcatcgtggaccggctgaagagcctgatcaaatacaagggctaccaggtagccccagccgaactggagagcatcctgctgcaacaccccaacatcttcgacgccggggtcgccggcctgcccgacgacgatgccggcgagctgcccgccgcagtcgtcgtgctggaacacggtaaaaccatgaccgagaaggagatcgtggactatgtggccagccaggttacaaccgccaagaagctgcgcggtggtgttgtgttcgtggacgaggtgcctaaaggactgaccggcaagttggacgcccgcaagatccgcgagattctcattaaggccaagaagggcggcaagatcgccgtgtaagcggccgcaagcttcgggtggcatccctgtgacccctccccagtgcctctcctggccctggaagttgccactccagtgcccaccagccttgtcctaataaaattaagttgcatcattttgtctgactaggtgtccttctataatattatggggtggaggggggtggtatggagcaaggggcaagttgggaagacaacctgtagggcctgcggggtctattgggaaccaagctggagtgcagtggcacaatcttggctcactgcaatctccgcctcctgggttcaagcgattctcctgcctcagcctcccgagttgttgggattccaggcatgcatgaccaggctcagctaatttttgtttttttggtagagacggggtttcaccatattggccaggctggtctccaactcctaatctcaggtgatctacccaccttggcctcccaaattgctgggattacaggcgtgaaccactgctcccttccctgtccttcggtctagaaggaacccctagtgatggagttggccactccctctctgcgcgctcgctcgctcactgaggccgggcgaccaaaggtcgcccgacgcccgggctttgcccgggcggcctcagtgagcgagcgagcgcgcagagagggagtgg

SEQ ID NO: 52 - DNA, 3569 bp, synthetic construct
  source 1..3569: mol_type = other DNA
acttacggtaaatggcccgcctggctgaccgcccaacgacccccgcccattgacgtcaataatgacgtatgttcccatagtaacgccaatagggactttccattgacgtcaatgggtggagtatttacggtaaactgcccacttggcagtacatcaagtgtatcatatgccaagtccgccccctattgacgtcaatgacggtaaatggcccgcctggcattatgcccagtacatgaccttacgggactttcctacttggcagtacatctacgtattagtcatcgctattaccatgctgatgcggttttggcagtacaccaatgggcgtggatagcggtttgactcacggggatttccaagtctccaccccattgacgtcaatgggagtttgttttggcaccaaaatcaacgggactttccaaaatgtcgtaataaccccgccccgttgacgcaaatgggcggtaggcgtgtacggtgggaggtctatataagcagagctcgtttagtgaaccgtcagatcgcctggagaggccatccacgctgttttgacctccatagtggacaccgggaccgatccagcctccgcgtctcaggggagatctcgtttagtgaaccgtcagatcctcactctcttccgcatcgctgtctgcgagggccagctgttgggctcgcggttgaggacaaactcttcgcggtctttccagtactcttggatcggaaacccgtcggcctccgaacggtactccgccaccgagggacctgagcgagtccgcatcgaccggatcggaaaacctctcgagaaaggcgtctaaccagtcacagtcgcaaggtaggctgagcaccgtggcgggcggcagcgggtggcggtcggggttgtttctggcggaggtgctgctgatgatgtaattaaagtaggcggtcttgagacggcggatggtcgaggtgaggtgtggcaggcttgagatccagctgttggggtgagtactccctctcaaaagcgggcattacttctgcgctaagattgtcagtttccaaaaacgaggaggatttgatattcacctggcccgatctggccatacacttgagtgacaatgacatccactttgcctttctctccacaggtgtccactcccaggtccaagtttaaacgccgccaccatggtgtcatactgggatactggagtcttgctttgtgccctgctgtcctgcctcctcctgactggctccagctcgggctcagataccggtcgccccttcgtggagatgtactccgagatcccggaaattatccacatgactgaggggcgcgaacttgtgatcccctgccgggtcaccagcccgaacattactgtgactttgaagaagttccccctggacaccctgattccggatgggaagagaattatctgggattcacggaagggattcatcatcagcaacgcgacctacaaggaaattggcctcctcacttgcgaagccactgtgaacggacacttgtacaagaccaactacctgacccaccgccagaccaacaccatcatcgacgtcgtcctgtccccttcgcacgggatcgagctctcggtgggagagaagttggtgcttaactgcaccgcccggacggaactgaatgtgggaatcgacttcaactgggaatacccgtccagcaagcatcagcataagaagctggtgaaccgggacctcaagactcagtccggcagcgaaatgaagaagttcctgtcgaccctcactattgacggagtgaccagatccgaccagggcctctacacttgcgccgcttccagcggactcatgaccaagaagaacagcactttcgtgagggtgcatgagaaggacaagacccacacgtgtccgccgtgcccagccccagagctgctgggaggcccttccgtgttcctgtttccgcccaagccaaaggataccctgatgatctcaaggacccctgaggtcacatgcgtcgtggtggatgtgtcgcacgaggaccctgaagtcaaattcaattggtatgtggacggagtggaagtccacaacgcgaaaaccaagccgagagaagaacagtacaattccacctaccgggtggtgtcggtgctgactgtgctgcaccaggactggctcaacggaaaggagtacaagtgcaaggtgtccaacaaggctctgcccgcacctattgaaaagaccatctccaaggccaagggtcaacctcgcgagcctcaggtgtacactctgcctccaagccgggacgaactgactaagaaccaagtctctctgacctgtttggtgaagggcttctacccgtcagacatcgcagtggagtgggagtcaaacggtcagccggagaacaactacaaaacaaccccccccgtgctggactccgacggctccttcttcctgtactccaagcttaccgtggataagagccgctggcaacagggcaacgtgttttcctgctccgtcatgcacgaagccctgcacaaccattatacccagaagtccctgtcgctgtcccccgggaaatagtgactgttctcatcacatcatatcaaggttatataccatcaatattgccacagatgttacttagccttttaatatttctctaatttagtgtatatgcaatgatagttctctgatttctgagattgagtttctcatgtgtaatgattatttagagtttctctttcatctgttcaaatttttgtctagttttattttttactgatttgtaagacttctttttataatctgcatattacaattctctttactggggtgttgcaaatattttctgtcattctatggcctgacttttcttaatggttttttaattttaaaaataagtcttaatattcatgcaatctaattaacaatcttttctttgtggttaggactttgagtcataagaaatttttctctacactgaagtcatgatggcatgcttctatattattttctaaaagatttaaagttttgccttctccatttagacttataattcactggaatttttttgtgtgtatggtatgacatatgggttcccttttattttttacatataaatatatttccctgtttttctaaaaaagaaaaagatcatcattttcccattgtaaaatgccatatttttttcataggtcacttacatatatcaatgggtctgtttctgagctctactctattttatcagcctcactgtctatccccacacatctcatgctttgctctaaatcttgatatttagtggaacattctttcccattttgttctacaagaatatttttgttattgtctttgggctttctatatacattttgaaatgaggttgacaagttacctaggaaaactgtcttcctgcccgggtggcatccctgtgacccctccccagtgcctctcctggccctggaagttgccactccagtgcccaccagccttgtcctaataaaattaagttgcatcattttgtctgactaggtgtccttctataatattatggggtggaggggggtggtatggagcaaggggcccaagttgggaagaaacctgtagggcctgcg

SEQ ID NO: 53 - protein, 20 aa, synthetic construct
ACCAAGCCGAGAGAAGAACA

SEQ ID NO: 54 - DNA, 20 bp, synthetic construct
  source 1..20: mol_type = other DNA
tgttggacaccttgcacttg

SEQ ID NO: 55 - DNA, 20 bp, synthetic construct
  source 1..20: mol_type = other DNA
cagcaccgacaccacccggt

SEQ ID NO: 56 - DNA, 3050 bp, synthetic construct
  source 1..3050: mol_type = other DNA
acgcgtctagttattaatagtaatcaattacggggtcattagttcatagcccatatatggagttccgcgttacataacttacggtaaatggcccgcctggctgaccgcccaacgacccccgcccattgacgtcaataatgacgtatgttcccatagtaacgccaatagggactttccattgacgtcaatgggtggagtatttacggtaaactgcccacttggcagtacatcaagtgtatcatatgccaagtacgccccctattgacgtcaatgacggtaaatggcccgcctggcattatgcccagtacatgaccttatgggactttcctacttggcagtacatctacgtattagtcatcgctattaccatggtgatgcggttttggcagtacatcaatgggcgtggatagcggtttgactcacggggatttccaagtctccaccccattgacgtcaatgggagtttgttttggcaccaaaatcaacgggactttccaaaatgtcgtaacaactccgccccattgacgcaaatgggcggtaggcgtgtacggtgggaggtctatataagcagagctcgtttagtgaaccgtcagatcgcctggagacgccatccacgctgttttgacctccatagaagacaccgggaccgatccagcctccgcggattcgaatcccggccgggaacggtgcattggaacgcggattccccgtgccaagagtgacgtaagtaccgcctatagagtctataggcccacaaaaaatgctttcttcttttaatatacttttttgtttatcttatttctaatactttccctaatctctttctttcagggcaataatgatacaatgtatcatgcctctttgcaccattctaaagaataacagtgataatttctgggttaaggcaatagcaatatttctgcatataaatatttctgcatataaattgtaactgatgtaagaggtttcatattgctaatagcagctacaatccagctaccattctgcttttattttatggttgggataaggctggattattctgagtccaagctaggcccttttgctaatcatgttcatacctcttatcttcctcccacagctcctgggcaacgtgctggtctgtgtgctggcccatcactttggcaaagaattgggataattactagatcgccaccatggtgtcatactgggatactggagtcttgctttgtgccctgctgtcctgcctcctcctgactggctccagctcgggctctgacacaggcagaccctttgtggaaatgtactctgagatccctgagatcatccacatgacagagggcagagagctggtcatcccctgcagagtgacaagccccaacatcacagtgaccctgaagaagttccctctggacacactgatccctgatggcaagagaatcatctgggacagcagaaagggcttcatcatcagcaatgccacctacaaagagattggcctgctgacctgtgaagccacagtgaatggccacctgtacaagaccaactacctgacacacagacagaccaacaccatcattgatgtggtgctgagccccagccatggcattgagctgtctgtgggagagaagctggtgctgaactgcacagccagaacagagctgaatgtgggcattgacttcaactgggagtaccccagcagcaagcaccagcacaagaaactggtcaacagggacctgaaaacccagagtggctctgagatgaagaaattcctgagcaccctgaccattgatggggtcaccagatctgaccagggcctgtacacatgtgctgccagctctggactgatgaccaagaaaaacagcacctttgtcagagtgcatgagaaggacaagacccacacctgtcctccatgtcctgcacctgagctgcttggaggcccctctgtgttcctgtttcctccaaagcctaaggacaccctgatgatcagcagaacacctgaagtgacctgtgtggtggtggatgtgtcccatgaggacccagaagtgaagttcaattggtatgtggatggggttgaagtgcacaatgccaagaccaagcctagagaggaacagtacaactccacctacagagtggtgtcagtgctgacagtgctgcaccaggactggctgaatggcaaagagtacaagtgcaaggtgtccaacaaggccctgcctgctcctattgagaaaaccatctccaaggccaagggccagcctagggaaccccaggtttacacactgccacctagcagggatgagctgacaaagaaccaggtgtccctgacctgcctggtcaagggcttctacccctctgacattgctgtggaatgggagagcaatggccagcctgagaacaactacaagacaacccctcctgtgctggactctgatggctcattcttcctgtacagcaagctgactgtggacaagagcagatggcagcagggaaatgtgttcagctgctctgtgatgcatgaggccctgcacaaccactacacccagaaaagcctgagcctgtctcctggcaagtgagcggccgcaagcttcgggtggcatccctgtgacccctccccagtgcctctcctggccctggaagttgccactccagtgcccaccagccttgtcctaataaaattaagttgcatcattttgtctgactaggtgtccttctataatattatggggtggaggggggtggtatggagcaaggggcaagttgggaagacaacctgtagggcctgcggggtctattgggaaccaagctggagtgcagtggcacaatcttggctcactgcaatctccgcctcctgggttcaagcgattctcctgcctcagcctcccgagttgttgggattccaggcatgcatgaccaggctcagctaatttttgtttttttggtagagacggggtttcaccatattggccaggctggtctccaactcctaatctcaggtgatctacccaccttggcctcccaaattgctgggattacaggcgtgaaccactgctcccttccctgtccttcgg

SEQ ID NO: 57 - protein, 12 aa, synthetic construct
AAARGDLATIAA

SEQ ID NO: 58 - protein, 12 aa, synthetic construct
AAARGDLGRLAA

SEQ ID NO: 59 - protein, 12 aa, synthetic construct
AAARGDLQNIAA

SEQ ID NO: 60 - protein, 12 aa, synthetic construct
AAARGDLQNLAA

SEQ ID NO: 61 - protein, 12 aa, synthetic construct
AAARGDLAAIAA

SEQ ID NO: 62 - protein, 12 aa, synthetic construct
AAARGDLATLAA

SEQ ID NO: 63 - protein, 12 aa, synthetic construct
AAARGDLATPAA

SEQ ID NO: 64 - protein, 12 aa, synthetic construct
AAARGDLGRPAA

SEQ ID NO: 65 - protein, 12 aa, synthetic construct
AAARGDLGTLAA

SEQ ID NO: 66 - protein, 12 aa, synthetic construct
AAARGDLARIAA

SEQ ID NO: 67 - protein, 12 aa, synthetic construct
AAARGSLQNIAA

SEQ ID NO: 68 - protein, 12 aa, synthetic construct
AAARGSLQNLAA

SEQ ID NO: 69 - protein, 9 aa, synthetic construct
AAARGSLAA

SEQ ID NO: 70 - protein, 747 aa, synthetic construct
MAADGYLPDWLEDTLSEGIRQWWKLKPGPPPPKPAERHKDDSRGLVLPGYKYLGPFNGLDKGEPVNEADAAALEHDKAYDRQLDSGDNPYLKYNHADAEFQERLKEDTSFGGNLGRAVFQAKKRVLEPLGLVEEPVKTAPGKKRPVEHSPVEPDSSSGTGKAGQQPARKRLNFGQTGDADSVPDPQPLGQPPAAPSGLGTNTMATGSGAPMADNNEGADGVGNSSGNWHCDSTWMGDRVITTSTRTWALPTYNNHLYKQISSQSGASNDNHYFGYSTPWGYFDFNRFHCHFSPRDWQRLINNNWGFRPKRLNFKLFNIQVKEVTQNDGTTTIANNLTSTVQVFTDSEYQLPYVLGSAHQGCLPPFPADVFMVPQYGYLTLNNGSQAVGRSSFYCLEYFPSQMLRTGNNFTFSYTFEDVPFHSSYAHSQSLDRLMNPLIDQYLYYLSRTNTPSGTTTQSRLQFSQAGASDIRDQSRNWLPGPCYRQQRVSKTSADNNNSEYSWTGATKYHLNGRDSLVNPGPAMASHKDDEEKFFPQSGVLIFGKQGSEKTNVDIEKVMITDEEEIRTTNPVATEQYGSVSTNLQRGNAAARGDLATIAARQAATADVNTQGVLPGMVWQDRDVYLQGPIWAKIPHTDGHFHPSPLMGGFGLKHPPPQILIKNTPVPANPSTTFSAAKFASFITQYSTGQVSVEIEWELQKENSKRWNPEIQYTSNYNKSVNVDFTVDTNGVYSEPRPIGTRYLTRNL

SEQ ID NO: 71 - protein, 747 aa, synthetic construct
MAADGYLPDWLEDTLSEGIRQWWKLKPGPPPPKPAERHKDDSRGLVLPGYKYLGPFNGLDKGEPVNEADAAALEHDKAYDRQLDSGDNPYLKYNHADAEFQERLKEDTSFGGNLGRAVFQAKKRVLEPLGLVEEPVKTAPGKKRPVEHSPVEPDSSSGTGKAGQQPARKRLNFGQTGDADSVPDPQPLGQPPAAPSGLGTNTMATGSGAPMADNNEGADGVGNSSGNWHCDSTWMGDRVITTSTRTWALPTYNNHLYKQISSQSGASNDNHYFGYSTPWGYFDFNRFHCHFSPRDWQRLINNNWGFRPKRLNFKLFNIQVKEVTQNDGTTTIANNLTSTVQVFTDSEYQLPYVLGSAHQGCLPPFPADVFMVPQYGYLTLNNGSQAVGRSSFYCLEYFPSQMLRTGNNFTFSYTFEDVPFHSSYAHSQSLDRLMNPLIDQYLYYLSRTNTPSGTTTQSRLQFSQAGASDIRDQSRNWLPGPCYRQQRVSKTSADNNNSEYSWTGATKYHLNGRDSLVNPGPAMASHKDDEEKFFPQSGVLIFGKQGSEKTNVDIEKVMITDEEEIRTTNPVATEQYGSVSTNLQRGNAAARGDLGRLAARQAATADVNTQGVLPGMVWQDRDVYLQGPIWAKIPHTDGHFHPSPLMGGFGLKHPPPQILIKNTPVPANPSTTFSAAKFASFITQYSTGQVSVEIEWELQKENSKRWNPEIQYTSNYNKSVNVDFTVDTNGVYSEPRPIGTRYLTRNL

SEQ ID NO: 72 - protein, 747 aa, synthetic construct
MAADGYLPDWLEDTLSEGIRQWWKLKPGPPPPKPAERHKDDSRGLVLPGYKYLGPFNGLDKGEPVNEADAAALEHDKAYDRQLDSGDNPYLKYNHADAEFQERLKEDTSFGGNLGRAVFQAKKRVLEPLGLVEEPVKTAPGKKRPVEHSPVEPDSSSGTGKAGQQPARKRLNFGQTGDADSVPDPQPLGQPPAAPSGLGTNTMATGSGAPMADNNEGADGVGNSSGNWHCDSTWMGDRVITTSTRTWALPTYNNHLYKQISSQSGASNDNHYFGYSTPWGYFDFNRFHCHFSPRDWQRLINNNWGFRPKRLNFKLFNIQVKEVTQNDGTTTIANNLTSTVQVFTDSEYQLPYVLGSAHQGCLPPFPADVFMVPQYGYLTLNNGSQAVGRSSFYCLEYFPSQMLRTGNNFTFSYTFEDVPFHSSYAHSQSLDRLMNPLIDQYLYYLSRTNTPSGTTTQSRLQFSQAGASDIRDQSRNWLPGPCYRQQRVSKTSADNNNSEYSWTGATKYHLNGRDSLVNPGPAMASHKDDEEKFFPQSGVLIFGKQGSEKTNVDIEKVMITDEEEIRTTNPVATEQYGSVSTNLQRGNAAARGDLQNIAARQAATADVNTQGVLPGMVWQDRDVYLQGPIWAKIPHTDGHFHPSPLMGGFGLKHPPPQILIKNTPVPANPSTTFSAAKFASFITQYSTGQVSVEIEWELQKENSKRWNPEIQYTSNYNKSVNVDFTVDTNGVYSEPRPIGTRYLTRNL

SEQ ID NO: 73 - protein, 747 aa, synthetic construct
MAADGYLPDWLEDTLSEGIRQWWKLKPGPPPPKPAERHKDDSRGLVLPGYKYLGPFNGLDKGEPVNEADAAALEHDKAYDRQLDSGDNPYLKYNHADAEFQERLKEDTSFGGNLGRAVFQAKKRVLEPLGLVEEPVKTAPGKKRPVEHSPVEPDSSSGTGKAGQQPARKRLNFGQTGDADSVPDPQPLGQPPAAPSGLGTNTMATGSGAPMADNNEGADGVGNSSGNWHCDSTWMGDRVITTSTRTWALPTYNNHLYKQISSQSGASNDNHYFGYSTPWGYFDFNRFHCHFSPRDWQRLINNNWGFRPKRLNFKLFNIQVKEVTQNDGTTTIANNLTSTVQVFTDSEYQLPYVLGSAHQGCLPPFPADVFMVPQYGYLTLNNGSQAVGRSSFYCLEYFPSQMLRTGNNFTFSYTFEDVPFHSSYAHSQSLDRLMNPLIDQYLYYLSRTNTPSGTTTQSRLQFSQAGASDIRDQSRNWLPGPCYRQQRVSKTSADNNNSEYSWTGATKYHLNGRDSLVNPGPAMASHKDDEEKFFPQSGVLIFGKQGSEKTNVDIEKVMITDEEEIRTTNPVATEQYGSVSTNLQRGNAAARGDLQNLAARQAATADVNTQGVLPGMVWQDRDVYLQGPIWAKIPHTDGHFHPSPLMGGFGLKHPPPQILIKNTPVPANPSTTFSAAKFASFITQYSTGQVSVEIEWELQKENSKRWNPEIQYTSNYNKSVNVDFTVDTNGVYSEPRPIGTRYLTRNL

SEQ ID NO: 74 - protein, 747 aa, synthetic construct
MAADGYLPDWLEDTLSEGIRQWWKLKPGPPPPKPAERHKDDSRGLVLPGYKYLGPFNGLDKGEPVNEADAAALEHDKAYDRQLDSGDNPYLKYNHADAEFQERLKEDTSFGGNLGRAVFQAKKRVLEPLGLVEEPVKTAPGKKRPVEHSPVEPDSSSGTGKAGQQPARKRLNFGQTGDADSVPDPQPLGQPPAAPSGLGTNTMATGSGAPMADNNEGADGVGNSSGNWHCDSTWMGDRVITTSTRTWALPTYNNHLYKQISSQSGASNDNHYFGYSTPWGYFDFNRFHCHFSPRDWQRLINNNWGFRPKRLNFKLFNIQVKEVTQNDGTTTIANNLTSTVQVFTDSEYQLPYVLGSAHQGCLPPFPADVFMVPQYGYLTLNNGSQAVGRSSFYCLEYFPSQMLRTGNNFTFSYTFEDVPFHSSYAHSQSLDRLMNPLIDQYLYYLSRTNTPSGTTTQSRLQFSQAGASDIRDQSRNWLPGPCYRQQRVSKTSADNNNSEYSWTGATKYHLNGRDSLVNPGPAMASHKDDEEKFFPQSGVLIFGKQGSEKTNVDIEKVMITDEEEIRTTNPVATEQYGSVSTNLQRGNAAARGDLAAIAARQAATADVNTQGVLPGMVWQDRDVYLQGPIWAKIPHTDGHFHPSPLMGGFGLKHPPPQILIKNTPVPANPSTTFSAAKFASFITQYSTGQVSVEIEWELQKENSKRWNPEIQYTSNYNKSVNVDFTVDTNGVYSEPRPIGTRYLTRNL

SEQ ID NO: 75 - protein, 747 aa, synthetic construct
MAADGYLPDWLEDTLSEGIRQWWKLKPGPPPPKPAERHKDDSRGLVLPGYKYLGPFNGLDKGEPVNEADAAALEHDKAYDRQLDSGDNPYLKYNHADAEFQERLKEDTSFGGNLGRAVFQAKKRVLEPLGLVEEPVKTAPGKKRPVEHSPVEPDSSSGTGKAGQQPARKRLNFGQTGDADSVPDPQPLGQPPAAPSGLGTNTMATGSGAPMADNNEGADGVGNSSGNWHCDSTWMGDRVITTSTRTWALPTYNNHLYKQISSQSGASNDNHYFGYSTPWGYFDFNRFHCHFSPRDWQRLINNNWGFRPKRLNFKLFNIQVKEVTQNDGTTTIANNLTSTVQVFTDSEYQLPYVLGSAHQGCLPPFPADVFMVPQYGYLTLNNGSQAVGRSSFYCLEYFPSQMLRTGNNFTFSYTFEDVPFHSSYAHSQSLDRLMNPLIDQYLYYLSRTNTPSGTTTQSRLQFSQAGASDIRDQSRNWLPGPCYRQQRVSKTSADNNNSEYSWTGATKYHLNGRDSLVNPGPAMASHKDDEEKFFPQSGVLIFGKQGSEKTNVDIEKVMITDEEEIRTTNPVATEQYGSVSTNLQRGNAAARGDLATLAARQAATADVNTQGVLPGMVWQDRDVYLQGPIWAKIPHTDGHFHPSPLMGGFGLKHPPPQILIKNTPVPANPSTTFSAAKFASFITQYSTGQVSVEIEWELQKENSKRWNPEIQYTSNYNKSVNVDFTVDTNGVYSEPRPIGTRYLTRNL

SEQ ID NO: 76 - protein, 747 aa, synthetic construct
MAADGYLPDWLEDTLSEGIRQWWKLKPGPPPPKPAERHKDDSRGLVLPGYKYLGPFNGLDKGEPVNEADAAALEHDKAYDRQLDSGDNPYLKYNHADAEFQERLKEDTSFGGNLGRAVFQAKKRVLEPLGLVEEPVKTAPGKKRPVEHSPVEPDSSSGTGKAGQQPARKRLNFGQTGDADSVPDPQPLGQPPAAPSGLGTNTMATGSGAPMADNNEGADGVGNSSGNWHCDSTWMGDRVITTSTRTWALPTYNNHLYKQISSQSGASNDNHYFGYSTPWGYFDFNRFHCHFSPRDWQRLINNNWGFRPKRLNFKLFNIQVKEVTQNDGTTTIANNLTSTVQVFTDSEYQLPYVLGSAHQGCLPPFPADVFMVPQYGYLTLNNGSQAVGRSSFYCLEYFPSQMLRTGNNFTFSYTFEDVPFHSSYAHSQSLDRLMNPLIDQYLYYLSRTNTPSGTTTQSRLQFSQAGASDIRDQSRNWLPGPCYRQQRVSKTSADNNNSEYSWTGATKYHLNGRDSLVNPGPAMASHKDDEEKFFPQSGVLIFGKQGSEKTNVDIEKVMITDEEEIRTTNPVATEQYGSVSTNLQRGNAAARGDLATPAARQAATADVNTQGVLPGMVWQDRDVYLQGPIWAKIPHTDGHFHPSPLMGGFGLKHPPPQILIKNTPVPANPSTTFSAAKFASFITQYSTGQVSVEIEWELQKENSKRWNPEIQYTSNYNKSVNVDFTVDTNGVYSEPRPIGTRYLTRNL

SEQ ID NO: 77 - protein, 747 aa, synthetic construct
MAADGYLPDWLEDTLSEGIRQWWKLKPGPPPPKPAERHKDDSRGLVLPGYKYLGPFNGLDKGEPVNEADAAALEHDKAYDRQLDSGDNPYLKYNHADAEFQERLKEDTSFGGNLGRAVFQAKKRVLEPLGLVEEPVKTAPGKKRPVEHSPVEPDSSSGTGKAGQQPARKRLNFGQTGDADSVPDPQPLGQPPAAPSGLGTNTMATGSGAPMADNNEGADGVGNSSGNWHCDSTWMGDRVITTSTRTWALPTYNNHLYKQISSQSGASNDNHYFGYSTPWGYFDFNRFHCHFSPRDWQRLINNNWGFRPKRLNFKLFNIQVKEVTQNDGTTTIANNLTSTVQVFTDSEYQLPYVLGSAHQGCLPPFPADVFMVPQYGYLTLNNGSQAVGRSSFYCLEYFPSQMLRTGNNFTFSYTFEDVPFHSSYAHSQSLDRLMNPLIDQYLYYLSRTNTPSGTTTQSRLQFSQAGASDIRDQSRNWLPGPCYRQQRVSKTSADNNNSEYSWTGATKYHLNGRDSLVNPGPAMASHKDDEEKFFPQSGVLIFGKQGSEKTNVDIEKVMITDEEEIRTTNPVATEQYGSVSTNLQRGNAAARGDLGRPAARQAATADVNTQGVLPGMVWQDRDVYLQGPIWAKIPHTDGHFHPSPLMGGFGLKHPPPQILIKNTPVPANPSTTFSAAKFASFITQYSTGQVSVEIEWELQKENSKRWNPEIQYTSNYNKSVNVDFTVDTNGVYSEPRPIGTRYLTRNL

SEQ ID NO: 78 - protein, 747 aa, synthetic construct
MAADGYLPDWLEDTLSEGIRQWWKLKPGPPPPKPAERHKDDSRGLVLPGYKYLGPFNGLDKGEPVNEADAAALEHDKAYDRQLDSGDNPYLKYNHADAEFQERLKEDTSFGGNLGRAVFQAKKRVLEPLGLVEEPVKTAPGKKRPVEHSPVEPDSSSGTGKAGQQPARKRLNFGQTGDADSVPDPQPLGQPPAAPSGLGTNTMATGSGAPMADNNEGADGVGNSSGNWHCDSTWMGDRVITTSTRTWALPTYNNHLYKQISSQSGASNDNHYFGYSTPWGYFDFNRFHCHFSPRDWQRLINNNWGFRPKRLNFKLFNIQVKEVTQNDGTTTIANNLTSTVQVFTDSEYQLPYVLGSAHQGCLPPFPADVFMVPQYGYLTLNNGSQAVGRSSFYCLEYFPSQMLRTGNNFTFSYTFEDVPFHSSYAHSQSLDRLMNPLIDQYLYYLSRTNTPSGTTTQSRLQFSQAGASDIRDQSRNWLPGPCYRQQRVSKTSADNNNSEYSWTGATKYHLNGRDSLVNPGPAMASHKDDEEKFFPQSGVLIFGKQGSEKTNVDIEKVMITDEEEIRTTNPVATEQYGSVSTNLQRGNAAARGDLGTLAARQAATADVNTQGVLPGMVWQDRDVYLQGPIWAKIPHTDGHFHPSPLMGGFGLKHPPPQILIKNTPVPANPSTTFSAAKFASFITQYSTGQVSVEIEWELQKENSKRWNPEIQYTSNYNKSVNVDFTVDTNGVYSEPRPIGTRYLTRNL

SEQ ID NO: 79 - protein, 747 aa, synthetic construct
MAADGYLPDWLEDTLSEGIRQWWKLKPGPPPPKPAERHKDDSRGLVLPGYKYLGPFNGLDKGEPVNEADAAALEHDKAYDRQLDSGDNPYLKYNHADAEFQERLKEDTSFGGNLGRAVFQAKKRVLEPLGLVEEPVKTAPGKKRPVEHSPVEPDSSSGTGKAGQQPARKRLNFGQTGDADSVPDPQPLGQPPAAPSGLGTNTMATGSGAPMADNNEGADGVGNSSGNWHCDSTWMGDRVITTSTRTWALPTYNNHLYKQISSQSGASNDNHYFGYSTPWGYFDFNRFHCHFSPRDWQRLINNNWGFRPKRLNFKLFNIQVKEVTQNDGTTTIANNLTSTVQVFTDSEYQLPYVLGSAHQGCLPPFPADVFMVPQYGYLTLNNGSQAVGRSSFYCLEYFPSQMLRTGNNFTFSYTFEDVPFHSSYAHSQSLDRLMNPLIDQYLYYLSRTNTPSGTTTQSRLQFSQAGASDIRDQSRNWLPGPCYRQQRVSKTSADNNNSEYSWTGATKYHLNGRDSLVNPGPAMASHKDDEEKFFPQSGVLIFGKQGSEKTNVDIEKVMITDEEEIRTTNPVATEQYGSVSTNLQRGNAAARGDLARIAARQAATADVNTQGVLPGMVWQDRDVYLQGPIWAKIPHTDGHFHPSPLMGGFGLKHPPPQILIKNTPVPANPSTTFSAAKFASFITQYSTGQVSVEIEWELQKENSKRWNPEIQYTSNYNKSVNVDFTVDTNGVYSEPRPIGTRYLTRNL

SEQ ID NO: 80 - protein, 747 aa, synthetic construct
MAADGYLPDWLEDTLSEGIRQWWKLKPGPPPPKPAERHKDDSRGLVLPGYKYLGPFNGLDKGEPVNEADAAALEHDKAYDRQLDSGDNPYLKYNHADAEFQERLKEDTSFGGNLGRAVFQAKKRVLEPLGLVEEPVKTAPGKKRPVEHSPVEPDSSSGTGKAGQQPARKRLNFGQTGDADSVPDPQPLGQPPAAPSGLGTNTMATGSGAPMADNNEGADGVGNSSGNWHCDSTWMGDRVITTSTRTWALPTYNNHLYKQISSQSGASNDNHYFGYSTPWGYFDFNRFHCHFSPRDWQRLINNNWGFRPKRLNFKLFNIQVKEVTQNDGTTTIANNLTSTVQVFTDSEYQLPYVLGSAHQGCLPPFPADVFMVPQYGYLTLNNGSQAVGRSSFYCLEYFPSQMLRTGNNFTFSYTFEDVPFHSSYAHSQSLDRLMNPLIDQYLYYLSRTNTPSGTTTQSRLQFSQAGASDIRDQSRNWLPGPCYRQQRVSKTSADNNNSEYSWTGATKYHLNGRDSLVNPGPAMASHKDDEEKFFPQSGVLIFGKQGSEKTNVDIEKVMITDEEEIRTTNPVATEQYGSVSTNLQRGNAAARGSLQNIAARQAATADVNTQGVLPGMVWQDRDVYLQGPIWAKIPHTDGHFHPSPLMGGFGLKHPPPQILIKNTPVPANPSTTFSAAKFASFITQYSTGQVSVEIEWELQKENSKRWNPEIQYTSNYNKSVNVDFTVDTNGVYSEPRPIGTRYLTRNL

SEQ ID NO: 81 - protein, 747 aa, synthetic construct
MAADGYLPDWLEDTLSEGIRQWWKLKPGPPPPKPAERHKDDSRGLVLPGYKYLGPFNGLDKGEPVNEADAAALEHDKAYDRQLDSGDNPYLKYNHADAEFQERLKEDTSFGGNLGRAVFQAKKRVLEPLGLVEEPVKTAPGKKRPVEHSPVEPDSSSGTGKAGQQPARKRLNFGQTGDADSVPDPQPLGQPPAAPSGLGTNTMATGSGAPMADNNEGADGVGNSSGNWHCDSTWMGDRVITTSTRTWALPTYNNHLYKQISSQSGASNDNHYFGYSTPWGYFDFNRFHCHFSPRDWQRLINNNWGFRPKRLNFKLFNIQVKEVTQNDGTTTIANNLTSTVQVFTDSEYQLPYVLGSAHQGCLPPFPADVFMVPQYGYLTLNNGSQAVGRSSFYCLEYFPSQMLRTGNNFTFSYTFEDVPFHSSYAHSQSLDRLMNPLIDQYLYYLSRTNTPSGTTTQSRLQFSQAGASDIRDQSRNWLPGPCYRQQRVSKTSADNNNSEYSWTGATKYHLNGRDSLVNPGPAMASHKDDEEKFFPQSGVLIFGKQGSEKTNVDIEKVMITDEEEIRTTNPVATEQYGSVSTNLQRGNAAARGSLQNLAARQAATADVNTQGVLPGMVWQDRDVYLQGPIWAKIPHTDGHFHPSPLMGGFGLKHPPPQILIKNTPVPANPSTTFSAAKFASFITQYSTGQVSVEIEWELQKENSKRWNPEIQYTSNYNKSVNVDFTVDTNGVYSEPRPIGTRYLTRNL

SEQ ID NO: 82 - protein, 744 aa, synthetic construct
MAADGYLPDWLEDTLSEGIRQWWKLKPGPPPPKPAERHKDDSRGLVLPGYKYLGPFNGLDKGEPVNEADAAALEHDKAYDRQLDSGDNPYLKYNHADAEFQERLKEDTSFGGNLGRAVFQAKKRVLEPLGLVEEPVKTAPGKKRPVEHSPVEPDSSSGTGKAGQQPARKRLNFGQTGDADSVPDPQPLGQPPAAPSGLGTNTMATGSGAPMADNNEGADGVGNSSGNWHCDSTWMGDRVITTSTRTWALPTYNNHLYKQISSQSGASNDNHYFGYSTPWGYFDFNRFHCHFSPRDWQRLINNNWGFRPKRLNFKLFNIQVKEVTQNDGTTTIANNLTSTVQVFTDSEYQLPYVLGSAHQGCLPPFPADVFMVPQYGYLTLNNGSQAVGRSSFYCLEYFPSQMLRTGNNFTFSYTFEDVPFHSSYAHSQSLDRLMNPLIDQYLYYLSRTNTPSGTTTQSRLQFSQAGASDIRDQSRNWLPGPCYRQQRVSKTSADNNNSEYSWTGATKYHLNGRDSLVNPGPAMASHKDDEEKFFPQSGVLIFGKQGSEKTNVDIEKVMITDEEEIRTTNPVATEQYGSVSTNLQRGNAAARGSLAARQAATADVNTQGVLPGMVWQDRDVYLQGPIWAKIPHTDGHFHPSPLMGGFGLKHPPPQILIKNTPVPANPSTTFSAAKFASFITQYSTGQVSVEIEWELQKENSKRWNPEIQYTSNYNKSVNVDFTVDTNGVYSEPRPIGTRYLTRNL

SEQ ID NO: 83 - protein, 735 aa, synthetic construct
MAADGYLPDWLEDTLSEGIRQWWKLKPGPPPPKPAERHKDDSRGLVLPGYKYLGPFNGLDKGEPVNEADAAALEHDKAYDRQLDSGDNPYLKYNHADAEFQERLKEDTSFGGNLGRAVFQAKKRVLEPLGLVEEPVKTAPGKKRPVEHSPVEPDSSSGTGKAGQQPARKRLNFGQTGDADSVPDPQPLGQPPAAPSGLGTNTMATGSGAPMADNNEGADGVGNSSGNWHCDSTWMGDRVITTSTRTWALPTYNNHLYKQISSQSGASNDNHYFGYSTPWGYFDFNRFHCHFSPRDWQRLINNNWGFRPKRLNFKLFNIQVKEVTQNDGTTTIANNLTSTVQVFTDSEYQLPYVLGSAHQGCLPPFPADVFMVPQYGYLTLNNGSQAVGRSSFYCLEYFPSQMLRTGNNFTFSYTFEDVPFHSSYAHSQSLDRLMNPLIDQYLYYLSRTNTPSGTTTQSRLQFSQAGASDIRDQSRNWLPGPCYRQQRVSKTSADNNNSEYSWTGATKYHLNGRDSLVNPGPAMASHKDDEEKFFPQSGVLIFGKQGSEKTNVDIEKVMITDEEEIRTTNPVATEQYGSVSTNLQRNGRQAATADVNTQGVLPGMVWQDRDVYLQGPIWAKIPHTDGHFHPSPLMGGFGLKHPPPQILIKNTPVPANPSTTFSAAKFASFITQYSTGQVSVEIEWELQKENSKRWNPEIQYTSNYNKSVNVDFTVDTNGVYSEPRPIGTRYLTRNL

SEQ ID NO: 84 - DNA, 60 bp, synthetic construct
  source 1..60: mol_type = other DNA
agcggctattgtagccagatcacctctggcagcagcgttgcctctctggaggttggtaga

SEQ ID NO: 85 - DNA, 60 bp, synthetic construct
  source 1..60: mol_type = other DNA
gctgctgccagaggtgatctggctacaatagccgctagacaagcagctaccgcagatgtc

SEQ ID NO: 86 - DNA, 63 bp, synthetic construct
  source 1..63: mol_type = other DNA
tgcagcgaggcgtcccaaatctcctctggctgcagcgttgcctctctggaggttggtagatac

SEQ ID NO: 87 - DNA, 63 bp, synthetic construct
  source 1..63: mol_type = other DNA
gctgcagccagaggagatttgggacgcctcgctgcaagacaagcagctaccgcagatgtcaac

SEQ ID NO: 88 - DNA, 65 bp, synthetic construct
  source 1..65: mol_type = other DNA
tgctgcaatattctgcaaatcacctcgggcagcggcgttgcctctctggaggttggtagatacag

SEQ ID NO: 89 - DNA, 65 bp, synthetic construct
  source 1..65: mol_type = other DNA
gccgctgcccgaggtgatttgcagaatattgcagcaagacaagcagctaccgcagatgtcaacac

SEQ ID NO: 90 - DNA, 65 bp, synthetic construct
  source 1..65: mol_type = other DNA
agctgccaaattctggaggtcacctcttgccgcagcgttgcctctctggaggttggtagatacag

SEQ ID NO: 91 - DNA, 65 bp, synthetic construct
  source 1..65: mol_type = other DNA
gctgcggcaagaggtgacctccagaatttggcagctagacaagcagctaccgcagatgtcaacac

SEQ ID NO: 92 - DNA, 65 bp, synthetic construct
  source 1..65: mol_type = other DNA
ggcggcaattgctgccagatcacctctggctgcagcgttgcctctctggaggttggtagatacag

SEQ ID NO: 93 - DNA, 65 bp, synthetic construct
  source 1..65: mol_type = other DNA
gctgcagccagaggtgatctggcagcaattgccgccagacaagcagctaccgcagatgtcaacac

SEQ ID NO: 94 - DNA, 65 bp, synthetic construct
  source 1..65: mol_type = other DNA
cgctgccagggttgccaagtcgcctcttgcagctgcgttgcctctctggaggttggtagatacag

SEQ ID NO: 95 - DNA, 67 bp, synthetic construct
  source 1..67: mol_type = other DNA
gcagctgcaagaggcgacttggcaaccctggcagcgagacaagcagctaccgcagatgtcaacacac

SEQ ID NO: 96 - DNA, 65 bp, synthetic construct
  source 1..65: mol_type = other DNA
ggcggctggcgttgccaaatcacccctagcagccgcgttgcctctctggaggttggtagatacag

SEQ ID NO: 97 - DNA, 65 bp, synthetic construct
  source 1..65: mol_type = other DNA
gcggctgctaggggtgatttggcaacgccagccgccagacaagcagctaccgcagatgtcaacac

SEQ ID NO: 98 - DNA, 65 bp, synthetic construct
  source 1..65: mol_type = other DNA
agctgcgggtctacccaaatcaccgcgggctgctgcgttgcctctctggaggttggtagatacag

SEQ ID NO: 99 - DNA, 65 bp, synthetic construct
  source 1..65: mol_type = other DNA
gcagcagcccgcggtgatttgggtagacccgcagctagacaagcagctaccgcagatgtcaacac

SEQ ID NO: 100 - DNA, 65 bp, synthetic construct
  source 1..65: mol_type = other DNA
cgcagcaagtgtaccaaggtctcctctggctgctgcgttgcctctctggaggttggtagatacag

SEQ ID NO: 101 - DNA, 67 bp, synthetic construct
  source 1..67: mol_type = other DNA
gcagcagccagaggagaccttggtacacttgctgcgagacaagcagctaccgcagatgtcaacacac

SEQ ID NO: 102 - DNA, 65 bp, synthetic construct
  source 1..65: mol_type = other DNA
tgctgcaatccttgcgaggtcacctcttgcagccgcgttgcctctctggaggttggtagatacag

SEQ ID NO: 103 - DNA, 65 bp, synthetic construct
  source 1..65: mol_type = other DNA
gcggctgcaagaggtgacctcgcaaggattgcagcaagacaagcagctaccgcagatgtcaacac

SEQ ID NO: 104 - DNA, 65 bp, synthetic construct
  source 1..65: mol_type = other DNA
agcggctatattttgcaggctgcctctcgcagcagcgttgcctctctggaggttggtagatacag

SEQ ID NO: 105 - DNA, 65 bp, synthetic construct
  source 1..65: mol_type = other DNA
gctgctgcgagaggcagcctgcaaaatatagccgctagacaagcagctaccgcagatgtcaacac

SEQ ID NO: 106 - DNA, 65 bp, synthetic construct
  source 1..65: mol_type = other DNA
ggcagccagattttggagagatcctcgtgctgctgcgttgcctctctggaggttggtagatacag

SEQ ID NO: 107 - DNA, 65 bp, synthetic construct
  source 1..65: mol_type = other DNA
gcagcagcacgaggatctctccaaaatctggctgccagacaagcagctaccgcagatgtcaacac

SEQ ID NO: 108 - DNA, 66 bp, synthetic construct
  source 1..66: mol_type = other DNA
tgccgcaagactgcccctagcagcggcgttgcctctctggaggttggtagatacagaaccatactg

SEQ ID NO: 109 - DNA, 64 bp, synthetic construct
  source 1..64: mol_type = other DNA
gccgctgctaggggcagtcttgcggcaagacaagcagctaccgcagatgtcaacacacaaggcg

SEQ ID NO: 110 - DNA, 45 bp, synthetic construct
  source 1..45: mol_type = other DNA
cggtagctgcttgtctgccgtttctctggaggttggtagatacag

SEQ ID NO: 111 - DNA, 42 bp, synthetic construct
  source 1..42: mol_type = other DNA
aacctccagagaaacggcagacaagcagctaccgcagatgtc